European Patent Application EP 4 790 135 A1, published August 12, 2026. Title: Retinal organoids. Applicant: UNIVERSITE DE STRASBOURG. The sequence listing filed with the application follows.

SEQUENCE LISTING (1 sequence)

SEQ ID NO: 1 - DNA, 123016 bp, Homo sapiens
  source 1..123016: mol_type = genomic DNA
ataataggagcgcttggcctctgagactacccggcagaagggacgtccccaaatgacactcggaggccgcctccctgggctccggtgctcggtgccgggaggagcggcacggctttctaccccgcctcaggtgcgccagcacgttttctgggcagcatctgtgtgttaggcgaccggagaggtgggttccttatagggaataagaaaactgaaactgacttccaactgcaggcagaaggaagcagtggtcattgctggaggttaaaactgttctgaccgggcgcagtggctcacgcctgtattcccagcactttgggaggctgaggcgagcagatcacgaagtcaggagatcaagaccatcctggccaacaaggtgaaaccccggctctactaaaaatacaaaaattagctgggcgtggtggcgcgcgccggaagtcccagctacttgggaggatgaggcagaagaatcgcttgaacccgggaggcggaggttgcggtgagccgagatcgcgccattgcactccagcctggcgactcagcgatactccgtccccctctccccgccccaagaaaaatctgttcagtggggagcgacaaggaaggagctttcagcccgactggggtcgcagggaagaattcaagatggcgtgtttaggagctctagctccttgacaaattagtaaaatgttagtcttaggagaagaacgaaaaggctctcctaggctaagaaacagcatacacagtgagaaacctcagaagaaataaaattcaaggaagatagcaacaacgaaaacatcagaaggaacactaaaggtataaaaagggcaaagacagccctagggttgggagggatccaggttttttatgaaaattagtggaatccctaaggtacttacctttgtattataagtatttgcatgtctccttctagaaacgtttatcactctgtgttacacagaccagcagtgttggcgtcaactgggagcctgttagaaatgcagaatcaggccccatccccagggttctgaatctgcattttaacaagatcacattaaagtgtgtgagaagcaatgctttgacagctggcagagagcagatccagatttgataccttttcatattctgcatgtaccttatacagagtaggcttttgcatttgcggaatgaaggatacaggaatactgtttactgtaatccatttctaaccagatatgccacttaggcttaaacacggccaatgatggggaaccccaagttacataggccaccctttctgagtgagcagctctatttgctgaaacgttcatttttatattatgaagttgacatcccacttaagtacaacaaattcactactcccctattctttgctctgcctcttataaactcattctttggctcataaaccaaagacagtttacaggaagaaaaaaaaaaggtacgattttactgcaacttcttgctcacccctccaaaatctttatgtctgagtacatgctttttggttatccctacttttctccctccacccctcaattccttaccataggacactgaagcaaggcccttgaagatacataatacattaaaccttgacttgtgtagtattcagttttctgaccccaaggtggtttcaccatgccaaataatatgtccttggtatgtatttccttgcagtagtcaaatcagcctagcagaaacaaagtacgttaaccaatggaaaactgacggagagaaataaactgtttttgcacagctaaatggaaatgacttttgaattatctgctttggaagattatccatgacactgttctgccctgctctgctctaacaacatttgtaagtcactcaacagttaataataaaagtcagttttgaatattgcaggttttagacacagaacaaatgtaatgtgacactgtaggaagaatgaattctccttagtcccaaattccttttttttttcttagattcgggaataagtaaagatacaagatcctcttaaccagtatcagtataattgttccctttagatttattgctgtcaccccaatgctcttctttctttctagaggaaaggaaaagaaggaggtaataggaaaagtaatgggttgtcctgatgttactgtgtctaggatgtcattgccactggtctcctcagatcaatcattctgcctaataaacagaaaaataacatgggcagcctcacatgcaagcctttacacacactgctaaagagacctcgcttcctctgagaagtgaggatgtgagaatgaaggattgattttacagaactggatgacaggttaaattgggcatctggaggtttatattcccatctccactcaccaagtttcatcctccatttatgaccaaggataggtataacatctgatcttgatggttactgtttcaaaaaacaatctgatcttttttataaagttaaacatttacttaatcatgcagcatactaattcccactcctgggtatttatccgagtgacataaaaacaagttcacacaaaacctgtaaacacatatatgtctttattcatataatagaaaaaacacaaaccctaaaatggaaaaaacataatgtccttcacctggtgatatggtttggttctgtgtccccacccaaatctcatctcaaattgtaatacccacgtgttgaaggaaggacctataaccttcacgtgtcaagggagggaagtgattggatgatgggggcggtttcccccatgctgttcttgtgatggtgcatgaattctcaccagagatgatggttttaaaagtgtttggcagttcttccttcattcacacacactcactgtctctcccctgtgccacataagatgagcttgcttcccttctaccataactgtaagtttctgaagtcctccccagccatgcagaactataagtaaattaaacctcttttctttataaattacctagtctcaggtatgtctttatagcagtgtgaaaataggctaatacatctggtgaatcaataattaaaatgtagcatagctataaatggaatactactcagtaataaaagaataactcgatacatacaataatattgatgaatctcaaatgcattatgggaagtaaaagaagccaggctccacttatgtgacattctggaaaaaggaagactatacggtcagaaaacagatcagtgtttgccaggacttgggggtggggggtggggagtgattgactacaaaagggcatgaagaaattttgaaggggaggtatggaacaggtctgtatcttgactgcagtggagttattgatacttaccaaactgtacaataaaaagtaaatttttattgtatgaaaattatgcctaaattaaaaactattaataaaatcagcattagcaaaatatatgagtttatacacaagagactactcaaccattgggtaaactaattatttttaaacaaataccattgattttaatctttttatagtttttatacaggcagagaaataatagtgattctgctcacctaaaggaagatagacccaattcaaaggtacagaattttccccaaatagtatcataatttttcctttcagattccaaaggatttgcatgtaaattctatcatgtgatcctcagaaccaccctatgagggtaagcagaacagatgatccatgatattccattttataaatgaggtgcaggttaaatatttagccagtatttcttgataagtatagtccatttatttcaacaaaccttgattgagggccccaatacttgttgagcttttgctgagccacccctgctctagaggagcacatgctctggaaatctctaaggaaactactacaactctaaatagatatggtgtatagtgatactgtgactaaatattcactgcaaatttcctctaaaattatagatatacattactggaataattagtatctcaacatcttcattaactatgaatctactatgtatatatcatcaccatgtgagtattaatttggtacaaataggctgccaactctaaaattatttgatgtagggcaagtacttttatctttttagccataaattttctcatctgtaaaatgagaggagtaggcatgtgatcattaaatcctgggttacggtaggaggcatcaatatgaaatgtttagcttaatatagatacagatgggtaaatatagaaatacttaaaaatgcatgtggattcatgtttaatacattagtatacacacatatatttccaagttctgtcctccgaaggcctagaagcaatgacaagcagaagcaaggagcacacccagcatccagttttttgtttctaatactgttctccaacaaagggaaccagagcccttgagaaaaatgcctaattctaggactggggcaggggatatacaagatgagtctgaaacatcttatagtgccagaaaataaacaagtgctttaaaaagacacaaaaaactgatggtatatcaaagtgacataggagccaactaaaagagctcccaatagctaaagctagaataattcaaaaaataagtaattcagcattggatttaacccaaattataaaataagatccatgagttcatactgatacaagtaaatgattgaagaaacaaataattgggagataattctcatattgaaaaattccaaaaaatttatgtactctaccctcgagaagatggaacataattctccaccccataagcatgagtcaagcctagtaaatgtttttcaaagagcgcagtatggaaaggaggaagaacactacctcaaccagctgatcaaggctaacatctctagtatgtcattagtggcatgtaaccttgatatgatatgatgagaatagcatttgatctttgatctgtttcctccccgaaactcattgccccagcctaatcatgaagaaatatcagacaatctcaaattaagtacaaaataaccagtactcttcagaactatcaaggccaccaaaaacaaggaaagtataagaaactgtcacagtctagaagagcctggtgatgactaaatgtaatgtgatatcctggatgggatcccaggacagaaaaagaacattaggttaaactaaatcaaacttgagtatgaaacttctttttttttaagtgcctaagtcctgaatgacaacaaaagactgaagaactgacaacgattagaggacactaaggagacttaacaactaaatgcaaaatgggaccctgaatctgatcctggaacacaaaaactaaattagtagaaaagtggtaaaataggtggtcgcgcgcccgaccgccgcagtcccagtcgagccgcgacccttccggctgcccccaccccacctcgccgccatgtgcctccgccgcccagcgctgttcccgggcgtggcgctgcttctcgccgcggcccgcctcgcggctgcctccgacgtgctaggactcagggacgacaacttggagagtcgcatctccgacacgggctctgcgggcctcatgctcgtcgagttcttcgccccctggtgtggacactgcaagagacttgctcctgagtatgaagctgcagctaccagattaaaaggaatagtcccattagcaaaggctgattgcactgccaacactaacacctgtaataaatatggagtcagtggatatccaaccctgaatatgtttagagatggtgaagaagcaggtgcttatgatggacctaggactgctgatggaattgtcagccacctgaagaagcaggcaggcccagcttcagtgcctctcaggactgaggaagaatttaagaaattcattagtgataaagatgcctctatagtaggttttttcgatgattcattcagtgaagctcactccgagttcctaaaagcagccagcaacttgagggataactaccgatttgcacatacgaatgttgagtctctggtgaacgagtatgatgataacggagatggtatcatcttatttcgtccttcacatctcactaacaagttggaggacaagactgtggcatatacagtgcaaaaaatgaccagtggcaaaattaaaaagtttatccaggaaaacatttttggtatctgccctcacatgacagaagacaataaagatttgatacagggcaaggacttacttattgcttactatgatgtggactatgaaaagaatgctaaaggttccaactactggagaaacagggtaatgatggtggcaaagaaattcctggatgctgggcacaaactcaactttgctgtagctagccgcaaaacctttagccatgaactttctgattttggcttggagagcactgctggagagattcctgttgttgctatcagaactgctaaaggagagaagtttgtcatgcaggaggatttctcgcgtgatgggaatgctctggagaggttcctgcaggattactttgatggcaatctgaagagatacctgaagtctgaacctatcccagagagcaatgatgggcctgtgaaggtagtggtagcagagaattttgatgaaatagtgaataatgaaaataaagatgtgctgattgaattttatgccccttggtgtggtcactgtaagaacctggagcccaagtataaagaacttggcgagaagctcagcaaagacctgaatatcgtcatagccaagatggatgccacagccaatgatgtgccttctccatatgaagtcagagttttcctaccatatacttctctccagccaacaagaagctaaatccaaagaaatatgaaggtggccatgaattaagtgattttattagctatctacaacgagaagctacaaacccccctgtaattcaagaagaaaaacccaagaagaagaaggcacaggaggatctctaaagcagtaggcaaacaccactttgtaaaaggactcttccaccagagatgggaaaaccactggggaggactaggacccatatgggaattattacgtctcagggccgagaggacagaatggatataatctgaatcctgttaaattttctctaagccatttcttagctgcactgttatggaaataccaggaccagtttatgtttgtggttttgggaaaaattattggtgttgggggaaatgttgtgggagtcgggttgagttgggggtattttctaatttttttgtgcatttggaacagtgacaataaataagacccctttaaactgtaaaaaaaaaaaaaataggaatgcggtccatggtttacttaatcgtataatatcagtgttcattttcttattttgataattgtcataatgttgtgtgaaatattctctttagggagcctgggaaagaatatataagaactctactatttttgtaacttttgtggaggactgcaatcatttctaaataaatagtcttaaaaataactaaagtaataaaaataataaagtacatgaggaagtccagtgtcatgttgtatagtcagaagattcttcaaatgagagaatttgcacccagggaaatagagaaaaaagactctgaaaagaactttttttgtttgtttggtttttgtgtttttttttgagacagagtcttgctctgttgccaggctggagttcattggcgcgatctcagctcactgcaacttccacctcccaggttcaagcaattctcctgcctcagcctcctgagtagctgggaccacaggtgtgtgccaccacgcctagtcaatctttgtactttttagtagagatggggtttcgccattccggccaggatggtttcgatctcttgacctcgtgatccacccgccttggcctcccagagtgctgggactacaggcatgagccactgcgtccggcctgaaaagagccttaaaataagtttatttaaaattctcagagaaaggaagatgccagtttgaacacaccccagctccatgccatttctcacccctacccacccaattttcacaagtcagaagctattggtactagcagataatagagtacaataaaggcctaaggatcagtgagcggcctgacagaacagatacaggtccacctctccttttgactaaatcaaactttaccatacatcaaaattatctagagggtcaaatatgcagattgctggtctgtgtacccagagtttctgattctgtaagtctggagtggggcctgaggacttgtgtcaagtacaaggctgatgtttctgcctcaagggccacattttgagaaacgcggcctagacaagggtctagagacgagtattcaagatccccagtaaacggcattgtgcagaaaggagtttgctgactcttagaaccgtaataatgcttcgccatacctaaaaaataaacaattaaaatcaactaggatgtgtgggaacaagtctctcatacagaattccaaataatttatgtagctattgccccctcaaggaattagagcacaactccatgcttgtgactgctttagcttgcaagtttggcccatgggtgggatttgggaacttggattttgggaggtttcttaccaccttaactgataagagtggctcacttttttaaaactgtttgtacaaacaatgtgatttatgctgaacacttgcttttcttctgggagtctggaattctgatatgtgctaagcagagggtgcctatgtgactagccccaactaaaaacctcatcacagagtgaagatatgtgaaagtctttcgattgtttccattttcttagaggaaaaaaagagaagatgattagctgactgtgaggaaaggagacaacatatttgaggtttgcggagataggttatatgcagtaatcaactagaaaggtgggacagagaattgtctagaaaaatgaagtatgattggcagtagcactgaaggtctacctatgttcagtggttatgaatttcagaaaaggcaagtcaccatactagtatttttctcttgtcatgtttagctgttttgatgcaggcagataaccaaaatgaagtttagctaagcaagtatggaggagagcaacaaagtaattgagagtgcgtggtagggtgtgattataatgttgggccatgcattttaaatgaggtgggctgggaaatgaagacagcaggttgatgggcagcccagtggagtcaaagaactgctggagttggagtaccagagtgaatgaactgaaaaggtaggagagagttttagagagtgggatgcttgaaattgagactttagtggtgttgcggttattcatgacaatgtcttagatatgtccatgtgggtataggtagttgagatgaggcagattataaaatcactggagtaagaagatcacataactaaaaggccagatagcagagtgttagagatctacctcaacattcattctctcttccttcttaataacagaaccttgatttttttcctgaggtattgcctctctgtataaagacacattttgtagtctccctagtagctagataagtaactaagttcttccaataagactaagtgaaaatgttatgtggaacttttgtaaagtctccttaaaagaaaaggggtgtgccattgttacatttctccttccttctgtgtagaatgtccatataatggctatagctacagtgggccatcttggaccatgaagtataaggtccacatgctgaagatagtggagcaaaaagagaagctgaagaactgttatatcatctcaggactatctacttccagacttttttaatataagaggaaaataaacttaaatcttatttaagtcattgttatttgaggtttttctgttaaatgtagctgaagctaatcctgactaagacattggattggtgaaagtattacctacatcagtgttaaaaccaactacaggagtagttttatattatagcgaggcagagagcttggtgctaaaatctttactgaatgaaggggagtcaacaattctgctaataatttcaatcagaagttatgggtgcgtcaaaggagctggggaatttgggaaagcaaggcagaacagcagtgaaatgagggtcaaggatgacatatatataccctaccttctttcttgtaccaagatcttggcttgttatgtcttatgtttgattgaggaaatgaattatagacgaggacatatcacttgtgttttaaaccacaactaaacattaaagataacataccaggccgggcgtggtggctcacacctgtaatcccagcactttgggaggccgaggtgggtggatcatgaggtcaggagatcgagaccatcctggctaacacgataaaaccccgtctctactaaaaatacaaagattagccaggcgtggtggcggacacctgtagtcccagctacatgggatgctgaggcaggagaatggcgtgaagccgggaagcagagcttgcagtgagccgagatggcgtcactgcactccagcctgggcgacagagcgagactctgtctcaaaaaaaaagataacatactgattcagatcaatgactcagaacagtttttggaagaacatgcttgtcctgcagacatttcaaaatgttaatcaccctttaatctcctttgtcactttttctaaaagaattattcactgtttgatttaatcctttaaaagtcatctatttacctcccatattgaatgtattcatttaattaattaattcttaacttactgaggtcttactatgtttcagccactacattaggcactaggaacacacagattaagtacaaaatgtattccttcgaggagtttactagttcaaggaggaaacaggtgagagaaccaaatattgttatatattatgataaggctattcataaaatgtaattgagaagaacactagttgtaatgagagcacagaggaaggtgacctatttgatactgagggtcaggaagatattccctgaagagaaaacagatgacctgaatctggacgatggtataggtgttagccagctgggccagtggagaatttatcaagaggaaagtacagcacaagaatgtgtataaaagcatggaaaaacttggcactcttagaaattccattaggcaatctggaggttgtttaaatgctgtattactcctaacaaaagtaacaggcccagtattaagtaaaataatcttatttatgaatgtacatgacatcaacatatcataaatttgctagtggggtctgctgggttaatgtgcacagcttcaataaagaacatatctaagtgattttaagaagttgtgtattttgactttatatcaccattttacattctctataattatagtctatacttactcagcaaaggaagcaaaactgctgaattaagttacattatgcattattaaagcaacttaatttgtggagaaatcatagaaaaacacagtaatttgaatgacttgtactagccagtattcctcctctgagaaaattctgccagaccatagctctgggtcaaatcctgagccaaaaaataataataataactccacatttctttttatttttaaattttataagagttttagatttaagaaaagttgcaaaaatagtacagcattctcatgtaccccacatccaatttcctttattgttgacattttacattcctctggtacatttgtcacaactaataaaccaatattgatacattattaaccaaaatgcatactttattaatattcccttaatttttacttaaagttctttttctgttgcaggagtccatccaggatactacattacatttagatgttatgtctccttaggcccctttattccgggacaatttctcagactttctttgttgatgatcttgacagttttgaggtagtcaggtatttgtagaatattcttcaacttgggtttgtctgatgtttttctcatggttagactgcattatggtttttgagaggaatacaacagagaggtaaagtggccttctcatcacttcatctcaaaggtacatactatcagtgtgacttattactgttagtgttaatcttgataacctagccgagatagtgtttatcagatttctccactacaaagttattttccccctttccatatgtaatttttggaaggaagtcactattcagctcacactagagaagtaggaagttctgctccatatccttgagggcagagttcataaattatttggaattcttcttcatgggagattcatctattctaccccatttattaatgtattcaattttctggcactacaagaatatatatatatttttgtaatcgactttaaaataattaggaaaatgatagaacattttaatataagaacaagatatggtaaattgatgaatattattagacattatcagtaacaagagctttgtatcttaagttgttttgagttcaatttcttgttcacatcttttagcttggttgagctaaaaaatcattaaccattgatttttttttgtaaccttgcatataatatgtacaatgagagaatcaattaatttagaattacatactcctaatttaaaaaagaaactggtgtacttattgctgataactaggaattatattatcaaagggctgttaattcaacaaatttacatgctaaaagagaaatttatatgttaaaagaaattaaaaggaagcaagagacattcaatttgcttttgatatgcagatttaaaaatactaggtccattttaatagatgataaatctccagtatcacaaggattagggaaagcaaaagacctgaaaagtaataccagttctcagttctctaactctcaaaaggcattccacaggtaaattcggtgaaagggccggcaattgttcaaatgtttaaataagaagaagttgtagttctcacatttccagttctcttacaggtgtgtgtatttggaaagataatactctctaatgttggtcttttccattgttcaggtttatcctgttgttaagtaataagcagcaatccaaatacaaacatattgtacaacagctattaatgaacatcacctgagttcagtgtgcctgacagctgacacttagttaatttctccatgaaacaagaacagtgaaacttccacagatgagaaaacagaatcatcagtggcactgggatgtaaacccaagtacctgctttgcatttcatttgctctgtttttcagaactacactttacgacatgagaaaaactggtataagcagaatgttcctacatttagttaatatcagttctaatttaatacataaatgacttgttcaaatacttacttagactccatgtaagggaggagaaaaggggagaaaattagagtgggggaagatgaatcaaatcacatttgtagaccacactacaacaattggaagctacttatcatatttcctaagataaagttttgttggatcctaatatgggaaggatttaaaagagatttaaaaaggtaggacagctaatttaaaatcccaaaattctcaaccaagttgatctcattggcagatggtagatgatctgaatgactgtgagcctagaaagttgaaagtaatttctttattgagaaaataaagacatggttcctaaggaaaagggctaaaaatgaccatgtttcaagtacactagtgaatagcaagtgaaacaaaatgtcttaagcatctatatgtcttatcttagatacatacaactattgtaggaacattatttctcttatctctcaggaaacatatttagttataatatgaaaaaaaactaaaattgagcttctaatagaaaatcaaaccctatcagaagaagagttacgtggagtaagcgattttataccgatgctgacttactctccctaccataaaatttgataaacaacaaacatttattaagcacctaccacatgtcaagaactctgctaaagacatacaaagatgactaaaagagtacctgagctcccagtctagggattaccacaaggaagagtgacggatcatgagtggaagggagatgagttaatacaaatggaaaacaggtttcattgtaggaaaaaggaaagtgaattaatgctttcgaaagagacattaaagtagatttctgggcaatatgaaactgagagtcaatctcgtcagattctgaaggcatctgtagataagcttcccaatgaaaaacagggcagtgacaataggacaactagaagtaagctataattatagcaaagaaggcaagagctagcataaacttgcctattgtcattgttgaagtcatagaactactcctttcaactactcttgtcatcagaggcttcctgatgcgatcatctgtggtgaggatagcttttcgagccccatcccactttccagggccctgtacacgatagtggattggagtgcagggtcccagtaataagtgtaatgccagcttggggtcagtgaaggccagagacagcagattgggcctgacccccaccaaatcagcaagctcttccatggtatctatgtagtctccctgaatggtatggcgttggctctccacatacctaaagtagaaaagacagaaaccatggcctgtcaataattcaatcagtcagtcaatcaattactgccttctgagtgcctgctattggctcaatatcagactaggagctgtggaatatagagaagaaagataaaacattggtcactgtccttaaggatcttaggacttacaaaaggagataagacagataaacatgaagcgagacttctgagtggtttcagactgccaaatagaaatgtggagaggggatagttaaaagagagctgtaatcgttaggttcttgaaggatgtgaaagatacagataagatgaggggcaggtatagcacatctagatacaaaggactctgatgttatgagaaagagaaaacccatcacaaaaattctcaagtatggcatcctctattatttgatgagggcagtggtgacagggtccacagggcaggacttcccagggccaatgttaatttggaatcctgaaaggatgagggagaatgatttattccacaagaggaagtagccctccaaatggagacaaatgaaattattacaccaagtgcagatttaaagatttaaaagggctttttaaaggggaaaatgtggttgattaacagtgatatctgtgtggtggagtgggatttggtgagctaatgagtgactttcactttttactttctgtaatgaaaagaaagaactgtaggacagagaggaagagaaaagccaagtcaagccaattgagattgaagaatccaagaacagggacaggaaaaaaatgatagaaaataaatttgaggtagaactggtgagatggaatttcagaggacctgatagagggtcaagtaggaatttattgaaatgggactagatttaggagagaaaaaggtaaaacagtaaagaatttgagagctttcccttatgaacaatatgttggctcaagagtttgtagacatgcatttatttatcctataatagtaggtcaagatctatactattcatgaggttgggcgtggtgtttcatgcctgtaatcctagcactttgggaggccgaggcaggcggatcactttgagctcaggagttcgagatcagcctgggcaacatggcgaaaccccatctctacagaaaacacaaaaattagctgggcgttgttagtatgcctgtagtcccagctactcaggaggctgaggcgggagaattgcttgactccaggaagtggaggttgcagtgagccaagatcacaccacttcactccagcctgggtaacagagtgagaccccatatcaaaaaaaaaaaaaaaaaaaaaagagctatagtattcatgaaggtttcacaaaagaggttcactagctcctgccttgattatgcagattaaataaactcatataaaacaatgtatacacatagtcggcctttaataaaggttacatgtatacatatgtaaaaaacctgcacgttgtacacatgtaccctagaacttaaatataaaataaataaataaataaatatttactatttcagaagttaaaaaaaaaaaaggttacattatatccttgggttactgactactcaggttcaggaggtggttagacaaaaataagtcaaaggaaagagaggaggaaagttaaaataagatactttagagccagaaaagaaagcactgcaagaaggaagaaatgtttaaaagcaccaaactcagtagtgagaagaaggaaaatgaagttggtcacaggtgacctttaagagagcagtttccggccaggtacggtggctcatgcctgtaatcccagcactttgggaggctgaggcgggcagatcacaaggtcaggagtttgagaccagcctggccaacatggagaaatcccatctctactaaaaatacaaaaatgagctgggtttggtggtgtgcacctgtagtcctagctactcaggaggctgaggcaggagaatcgcttgaacccaggaggcagaggttgcagtgagcgaagatcgtgccacttactccagcctgagtgacagagtgagactccgtctaaaaaaaaaaaaaggcagtttaaggagtaaggatggaagttaacaatgcagaaggcttagggaggcagcaaaaggtgagaatttagaaaatttagtgcagaggtttggcagtgaaaggaaggaggaaaataggagagcacctggaagttgtaacggaattaaataaaaacttactttctcctcctcccacacaaaggaaagttatgcaagtatcatcagttgaagataaccacctctttaggcctggaatgattgtgtctctcagttttccacagaaatttagagacttaccatcaatttccactttgtccaaataaaaaacacccagcgattgagcttaagttctgaaattcagactgctaaatgattgtgttcatcaaaacactaagcagctggctgttaccatgttcccaactcacagtgactattcataccatgagccactgtgacttgagtgtgctgtcacatgagcattgccagcaaagcggccactgcagacttgtaaatctacctacagatttgtaattcacccatagctacctctcattcatttactgtcactcttccttcctctggcaagtctactagcacttcaagtaatcctcacaaaaataatataccttctgccttctgattttatttccatatgcattttcctatgtgactttttttaggcattaaacatatgattttagacacctaaaacttttctctcttttcttacccatatttagactactagtgctatttctccattctattgtcacaaattatttttccttttttcttcataatagaatctaaatccttaagctaacatgaggcagttaaatacagtacaatatttcttttattaagaaataagtagaaatgtaaccatatatcttcctgggagagtttcttaccttttgtcaatttcctcttgagctttagatatttctgccatcatttcactctgtgagggcaatgtctttagacctaaaaacaaaaattaacattttaactgtaaaattacctcagaaggaacaataatcctataaacaattactatgctatggagaattcaaagaaatacagggtaagtttcctgtactcaaggaggttacaattcacttgatcaccttaccaccaccacaatataatattaacatctgcagcttactctacttattcttctttgtctttggaagggatttcccctactctgacttccaaccaatacctgcctcctccctaatgtagtctttcagttgggaaatgaaatatggacatgagaaaatggacttaaaggtatatggaaaattagttacaaagttaaagggcaggggagtgggaaaacacagctgcacctgtattcttgataacaaagggaccttatatcaacagaaagagaatgaagtaaaaataaattttttgtttttattattataccttaagttttagggtacatgtgcacaatgtgcaggtttgttacatacgtatacatgtgccatgctggtgtgcagcacccattaactcgtcatttagcattaggtatatctcgtaatgctatccctccccactacccccaccccacaacagtccctggagtgtgatgttccccttcctgtgtccatctgttctgattgttcaattcccacctatgagtgagaacatgcggtgtttggttttttctccttgtgatagtttgctgagaatgatggtttccagtttaatccatgtccctacaaaggacatgaactcttcattttttatggctgcataatattccatggtgtatatgtgccacattttcttaatccagtctatcgttgttggacatttggcttggttccaagactttgctattgtgaatagtgccgcaataaacatacgtgtgcatgtgtctttatagcagcatgatttataatcctttgggtatatacccagtaatgggatggttgggtcaaatggtacttccagttctagattcctgaggaatcgccacagtgacttccacaatggttgaactagtttacagtcccaccaacagtgtaaaagtgttcctatttctccacatcctctccagcacctgttgtttcctgactttttaatgatcgccattctaactggtgtgagatggtatcccattgtggttttgatttgcatttctctgatggccagcgatgatgagaattttttcatgtattttttggctgcataaatgtcttcttttgagaagtgtctgttcatatcctttgcccactttttgatggggttgtttgtttttttcttataaacttgtttgagttcattgtagattctggatattagccctttgtcagatgagtaggttgtgaaaattttttcccattttcttggttgcctgttcactctgatggtagtttctttagtccatcttgaattgatttttgtataaggtgtaaggaagggatccagtttcagctttctacatatggctagccagttttcccagcaccatttattaaatagggaatcctttccccatttcttgtttttgtcaggtttgtcaaagatcagatggttgtagacatgcggcattatttctgagggctctgtcctgttccattgatctatatctcccttttggtaccagtaccatgctgttttggttactgtagccttgtagtatagtttgaagtcaggtagcgtgatgcctccagctttgttcttttggcttaggattgacttggtgatgcgggctcttttttggttccatatgaactttaaaatagttttttccaattctgtgaagaaagtcattggtcacttgatgcggatggcatttaatctataaattaccttgggcagtatggccattttcacgatattgattcttcctacccatgagcatggaatgttcttccatttctttgtatcctcttttatttcattgagcagtggtttgtatttctccttgaagaggtccttcacatcccttgtaagttggattcctaggtattttattctctttgaagcaattgtgaatgggagttcactcatgatttggctctctgtttgtctgttgttggtgtataagactgcttgtgatttttgtacattgattttgtatcctgagactttgctgaagttgctcatcagcttaaggagattttgggctgagacaatggggttttctagatatacaatcatgtcgtctgcaaacagggacaatttgacttcctcttttcctaatcgaataccctttatttccttctcctgcctaattgccctggccagaatatccaacactctgttgaataggagtggtgagagagggcatccctatcttgtgccagttttcaaagggaatgcttccagtttttgcccattcagtatgatattggctgtgggtttgtcataggtagctcttattattttcagatacatcccatcgatacctaatttattgagagtttttagcatgaagtgttgttgaattctgtcaaaggccttttctgcatctattgagataatcatgtggtttttgtcattggttctgtttatatgctggattacatttattgatttgtgtatgttgaaccagccttgcatcccagggatgaagcccacttgatcatggcagataagctttttgatgagctgctggattcagtttgccagtattttattgaggatttttgcatcaatgttcatcaaggatattggtctaaaattcttttttgttgtgtctctgccaggctttggtatcaggatgatgctggcctcataaaatgagttagggaagattccttctttttctattgattggaatagtttcagaaggaatggtaccagctcctctttgtacctctggtagaattcggctgtgaatccatctggtcctggactctttttggttggtaagctattgattattgccacaatttcagagcctgttattggtctattcagagattcagcttcttcctggtttagtcttgggagggtgtatgtgttgaggaatttatccgtttcttctagattttctagtttatttgtgtagaggtgtttatagtattctctgatggtagtttgtatttctgtgggatcggtggtgatatcccctttatcatttttactgcatctatttgattcttctcttttcttctttattagtcttgctagcagtttatcaattttgttgatcctttcaaaaaaccagctcctggattcattaattttttgaagggttttttgtgacttaatttccttcagttctgctctgattttagttatttcttgccttcttctagcttttgaatgtgtttgctcttgcttttctagttcttttaattgtgatgttagggtgtcaattttggatctttcctgctttctcttgtgggcatttagtgctataaatttccctctacacactgctttaaatgtgttccagagattctggtatgttgtgtctttgttcccattggtttcaaagaacatctttatttctgctttcgtttcgttatgtacccagtagtcattcaggagcaggttgttcagtttccatgtagttgagtggttttgagtgagttttttagtcctgagttctagtttcattgcactgtggtctgagagacagtttgttataatttctgttcttttacatttgctgaggagtgctttacttccaactatgtgatcaattttgcaataggtgtggtgtggtgctgaaaaaaatgtatattccgttgatttggggtggagagttctgtagatgtctattaggtctgcttggtgcagagctgagttcaattcctgggtatccttgttaaccttctgtctcgttgatctgtctaatgttgacagtggggtgttaaagtctcccattattattgcgtgggagtctaagtctctttgtaggtcactaaggacttgctttatgaatctgggtgctcctgcattgggtgcatatatatttaggatagttaggtcttcttgttgaattgatccctttaccattatttaatggccttctttgtctctttagatctttgctggtttaaagtctgttttatcagagactaggattgcaacccctgcctttttttgttttcgatttgcttggtagatcttcctccatccctttattttgagcctatgtgtgtctctgcacatgagatgggtttcctgaatacagcacactgttgggtcttgactctttatccaatttgccagtctgtgtattttaattggagcatttagcccatttacatttaaagttaatattgttatgtgtgaatttggttctgtgattatgatgttagctggttattttgcttgttagttgatgcagtttcttcctagccttgacagtctttacattttggcatgtttttgcagtggctggtaccggttgttcctttccatgtttagtgcttccttcaggagctcttttagagcaggcctggtggtcacaaaatctctcagcatttgcttgtctgtaaagtattttatgtctccttcacttatgaagcttagtttggctggatatgaaattctgggttgaaaattcttttctttaagaatgttgaatattggcccccactctcttctggcttgtagagttactgccgagagatctgctgttagtctgatgggcttccctttgtgggtaacccgacctttctctctggctgcccttaacattttttccttcatttcaactttggtgaatctgacaattatgtgtcttggagttgctcttcttgaggagtatctttgtggcgttctctgtatttcctgaatctgaatgttggcctgccttgctagattggggaagttctcctggataatatcctgcagagtgttttccaacttggttccattctccccgtcactttcaggttcaccaatccgacgtagatttggtcttttcacatagtcccatattccttggatgctttgttcgtttctttttattcttttttctctaaacttcccttctcacttcatttcattcctttcatcttccatcactgatatcctaccaaacccaaataatttttttttgtagttttagtagagacgaggtttcaccatattggtcaggctggtctcgaactcctgacctcagatgatccacccgtctctgcatcccaaggtgctgggattacaggcatgagccaccatgcccagccaaaataaatcttaatcacattttatgcctaaagtcctgtggaagataagcttcattttctaaacatgtttctttgataagagtaggggttaaggccaaggggaactcataatacctaatattaactgataaatttaagtaagatgcacaaacagttccagttgtaggaattatacaccaaggacagggctagactaaggcttaatagtatttaagccagtatgaacaatgctaagcttaaacaattagttgtatgcccctataactagggactatgccatgtagaagattttggccacatccagtcctaaggtgtcactccataaaattgtggaatatggaatttcagaatggcaatatattttacctgatacaagcattctttctacaagtactctaacctagtggttatctcattcctctttaaacatcactggtgatgggtatctataataattatatctgaggtgattatataattatttgactgctctggctgctggaacattattgtttttattgaccccaagatctgactctttgcatttgcaccactggaccaagctctgctttctggagccacagagtttaatgttaatacatgacagctcttgaaacatttggaaatgattgtcataactcctttaagtcttctcattatcaggctaaacagtacatgtttcccatataatggttttcacattctctgccatcttggttgcccttcactaagcatactctaataactatcctggtgtatccctcttaaaatatggaactcagaagttcatcactctcaaatagccttctgttgttttccatgtgtttttacattttagccatgggaattattatttatcatcataaatcaattaggaaacactgaaatgcttcatttaagcttaatcataggtctcttcggatactcaaaataagcgttttgagagtcaatttccaaattacttctacacaaccacaagttttacttctattagctagaaacatgaaggaggaggtatatttcttgattgtgggagacacccaattcataaaagaaagaaaaaaacaacaaaaaaccctatctattaccctatctgtctatatatagatagataaagaggtatatacatcttagtctagagctcatggggtgaaaaaatttaaaaaaattaaaaaattttaaaaagatgtatacatctttttacgtgtatactctgtggtacagttatgtcttaattcataaattttgtttttgcagtgtttccttatttagacacattagctttaccatatttcttatctccctccatgtctttgctccctgtcttagtttcccaattccaatgaatggcctcaacacctgaacagattcttttctgtctctcttctccaacatgctttctgtcaccaaattcttcagatttgcctgtgaaatttcatttaagtctggctcctccaattcctttagagtgtcattaccttggtttaaagctctcatgctgtcttactgagacttttaccacaggctcgtactgacctatttcccatttcactcctctctaacatatcttctaaactggagatctgatttgactcctcttccagttaaaatccttcagtggttctccaacttgtaccttaaatgcaaactcttgatattgcctgtgaatatttctagtttcattttccttcattcctataacactttaccagcattctgaactacttgcagttcccagaactctatttgttctgtcactttcatctaactttgcataaacagtagtgattatttcccctctatggtcaatatttccttgtccttttagtaaattcctatgtagttgtagggagaattgggtacttattgcccactgctctcatggcagctcttctgcattgctactggagcacttgtttaggatatagttaaatatctgctgaatgaacaaatcattaagcgtctgtttacttgtctgtctttgatatggtttggctgtgtccccacccaaatcttatcttgaattttgggtcccacaatccccatgtgtcatgggaggggcctggtgggaggtgatttaatcatggggtggttactctcatactgctcatgctgttctcatgatactgagtgagttctcacgagatctgatggttttatacggggctttccctttcactcagcactcattctctctcctgccaccctgtgaagaagttccttctgccatgattgtaagtttcctgaggcctccccagccatgcagaactgtgagtgaattaaacctctttcctttagaaactactcagcctcaggcagttctttatagcagcatgagaatgggctaacacagtcttccttgcttggctctgcattccagaaagatagggattttctgtatggtcatatttgcttctccagcccctagcagaaggcctggtacatactaaaaggtcagtatatgttatctgaagaatgttgaagaacagtgaggaactgaagttcagagatcttccaagggttccaagacaaggtgggaaggaagagagtctgaattagagttctgtggtggtaggccttcagtctgctgtcagcctaaagcaggttgtatctgtgtaatcctgacttgctcctgcatatttcagtgtatagctaatgttatgagagaaaagagatctggctcccattctgcaatttcagtccagttcaggcttttaacataactggaaattggctaaggtagcccataagctgagatcctcaaataagaagtttctacatcagaatttagaatttaatttacctcaaggctaaactgacatttcttagaatagatgtttattagatacctcttatgtgctaggcagtggtctaggcttgcaatacaaaggcaaataaacatgagtcctttacttaaggagctatcactatattacaaagggagggaagaaatatgcatagacttttcctatagaaataaaaagtaaaaggagggcatatcaagaagaaagcacagtggaagcaaaagcacagggtacaagggtacctgctgtgtttgctgcttagtgggtacgtcatccagtgcatctagagtattgtaggaagtatggtaaagactagtgaaagatgggcctgaggccgggtacagtgactcatgcctgtaatcccagcactttgggaggctgaggcaggcggatcacgaggtcaagagatggagaccatcctggctaacatggtgaaaccccgtctgtattaaaaacacaaaaaaactagccgggcatggtggcgggcgcctgtagtcccagctactggggaggctgaggcagtagaatggcctgaacccagaaggtggaacttgcagtgggccgagatagcgccactgcactccagcctgggcgacagagcgagactgcatctcaaaaaaaaaaaaaaaaaaaaaaaaagaaagaaagatgggcctgaaattggaggttgtatccaatttgtggaggaactttaatgccagcctatgacataatgacttcttgtgatccagagatttggtgtaacttgatatagttttgaaggaaagaaagttgctgagtgaaaataaaacacttgcaagggctgcaaaagacgcaatcaaaacagaaactatgtttcatttcagtcaaggcaaggaagtaaattcagtgttctagaaaagagtagaatattttcttgacaagagaacaataattccagagaacagaagaagaaggaaaatggggcttggtagggaacagacaaggaaggaggcaggctttgttgggcagacatgaaaaaaatgggaaaaacaagctaatccaaagggtttaaaattggcatagtgaagggataattcagggaagagaaaggcaagaatgtgggaggcagacagattggccatggacagaataaaaaacccagagttcctgttggaagtctggtaaagttagagaattctgaagatttcttccttccaggtgttagaaaaaagctggaggaattagcactaggcttctgctagcataggaagctgggctttttgtacattttccctaagatcccataatctcataaccataatgcagactcttgcaaatactcattttctctatttcctctcaagaattcacttggtcttggaaaagagtcccagttgcttaaagtatactaagatgctgtggcctgttttaatgaactgttctccgcttatgtaattgacccaattaaaagatcactttaatatgactagaattaggccaacttaatgggctatttgcgtttgactacttgtatagttctctcaggtagtacataatctgctggataggactggaagtaatagaaatttggggaaatttagaaaggttgttgaactatcaactgtaataccattggttctttttttctctgcaactgtgaagattttcactagtgaaaacaaaaaaggtgtaattccaacaggaactctgagtagttttaattaaatgctagtaacaatagcaaattttgttataacaaccatagaatcagtgaatttcttctttagaaggacccttaaacatcatcttgtttctctctatcctgaggcttgaatctactccataccttccccctctcctgccccggcccagtgagcattcagtcatttggcatccttttccttttctgcttagaatttcagaggcagctggttccatcatgaaatggcattggctgataggaaaaaggttttggatttttttcttaatggtaagctgatgtgtaaccctcaagatttcactccttgattctggtttgaccctttgaagctatactgagtaaatctaatccttcttccatgtgccttcccttcagatatttgaaggaaattctcatatctctcctgaagtttatcttctccaggctaaatctctctccggctttttcagttgtacttcagatggcatgttttcaaatcccttaaaaaatttttctctctctccttattaaacgcactccagcttcacttttaaaatgtatcattaggtgtggtctggccagtttagagaacaacagttgtaatgttctagaacattatagttttttaatgatgctagatttaattatttctttggaagctatatcattctactgactcatatgaaacctattcccctttttttttcatatattcctagccaaaactgaaagaggggacataaaaggagaaaagtgagaatttgggggattgaatatcctacaatattgactagtctgcaaccaggtcttaattttcggccgaaataaagtcatactatttctatattttatttttatctataatgaaagaagataaaactattttacttcagaaatatatgccagttgcctaaaatctagatgagtaaattctaatttggagtacacattggaattactggggaatatttttctcaaagatgttatgactgccccaccccagactaactaaataagcatcagcaaggatggtgtcaaagcatgcatagcttggaaaaatttcccaggtatgatgtatgtccatggttataaattgctactttagattcactcaaaaatatatttttctgtactaactttgtgctaggcactgttgtaatcatacatgctatctctagctatttaaaaacaagtacctaaacagaggtaaacatatcaccaagtaattaagtagtctatttgcatggtcacttacctttaaatacctgagtggcccagcgtccttggagctctgaaatgggcataatggctcctaagggctgaatcaagcctatgattgcaagagttggcctttccaggttaggagggaagacctttttatacagggatatcttgtttttgaccactttgacggaatcttccagaaatggaaagtcaaagctatagcctgtggcaaagataacagcatcaatgtcatcctccctggagccatcctcaaatatggcagctgtctccgtgaattccttcacatttcctttcactttcaccaagccagaaatgatacgatttggcaggtcatcatttaaggttggatgctgactcagagctctgtgagtcgtgacaaagatcaagtggagaaatgagagaaagagaaatcagtaccacataagtaaaattttgctttggtggaggtaaacaggatgccaataatcttccccttggtctatgcatgaagtttggaaaaggtctaatttatactaggttggcacagatcaagatcagatctgaagttggaccctggatgcactgaaagggagagtgttggaggagtgaaggaagagtgttgtttgaggagtgcatatatgatttctcaagtaacaataatattctgtgtgtgatatgataaggccacaggtcaatagtttgtattctcataccaagaagtctgacagaactaagctgtcaacattctgttcagtctcatttccagtttcaaaggctcaagagctaagtttaggccactgttttccaaactgtatgataaattacatgtatgtagcaatttacagtttataagttgcttttacatgcattaacttgactctcacaaaactctatgaaggaagcagaataggtgtcattatccaggttttataaatgagggaattgaggcctagaaaagttatgtgacttgtccaatgatacacagcctaggattttagaatttatctcaaagttgttttcagtgaattatcttggtatacttcgggcttgttattgtttcctagggacagcgtaggatacggatactggaaacattgggttggtgcaaaagtaattgcttatttttttgccattacttttaataataataaggctggtttctagtatcgtggagctttctaaaaagcagttctttttttttttttttttttttttgagacagagtctctacttcttttgccgaagctggagtgcagtggcatgatcttggctcactgcaacctccacctcccaggttcaagtgattctgctgtctcagcctcccgagtagcttggactacaggcacctgccaccatgcctggctaatttttgtatttttagtagagacagggtttcaccatgttggccaagctggtctcgaactcctgacctcgtgatcctcccacttcagcctcccaaagtgctgggattacaggcgtgagccacagcacctggcctaaaaagtagtcttaatgcctgaatactatattaactcatcttcagacagagctgtcctggcctcaggaattttatatgtttaaattaccactactggtttgttgcatttagttatgctttgacactaggtcgattgtgttctgcattccaacctcatgatttcatctttttctccaaacctactccttttcaccagcagtaccaccatccatccatatagttgcccaacccacaaaaccatgagttatatatctggtcaccaagccttttccctttctcctcttaacatccccaagatagttttatctactccttgttatctcaaccagatgatacaattgtctttaggacctcctgtctcatcccactcccacaccattttcaaaatggtctttctaaaatgtaggtatgattatgttactcacttgcctaaatctttgaatggctttggactgtcttcattccatactttttatttagtagaccaaaggtttccttttttttttttgacagtaacaatatgtttattataacatccagccaagaatacaaacacaaaatacctcttaatgtaaggagaataagaaaacatcacgcgattcttagaatactactacaaatacagccttcacctacagtaaaaattaagccaatttcaatcattttggtcatcatcccagtctttcttcccacttggaggcttgggcccaccatctggttttgccatgattacctgacccactctaagtacagtgactgcagcattagcagcgagtttgatagaccagtgttttcccaggtaagtatctagaacaccagcttccaacatgtccgttacagcagggactacagcctcagtatctaatccaacatttttatttccttcttgaggtactgcataaagtttagagattacttcattggccttaactccagagttttctccagagtatttctgccagtgcacggggaatagcttcaaacgcctcagcaaacttcttaatagcgtactgttcaagtccaggacatgtctctccatatgatgtgatctgtttggctaattcaatttctgttgctccacctctgggtacaagacgtttatcccttgtaagaactttgaaagtattaacaccatcatctactgccctttctatgtcatccatcagattgtctgtagagccccgaagtactatggtagaaatgatgccatcttccttttcatgcttaaaaaccaccacctgagtatctccaacttctgagaggtaaacactgtctcagtgtcccatttcttcaaggacaggaggtgtcaatctaggaagagctgtagcaccaactgttttacagagtcttcggacatcccattttgagtttagcttcactaacatcatattatatttgtttgcataatgaagagccatgtctgccactttgccacctgttactacaacatttgcaccagtatcagcaatagctttgacttatgcatccatgagattttcttctcccttacttaaattcatcaattcttcatcagtctttatcaacactgttcccttagtttctgttatcatgccatcaaaaggacaagagtacactgctatttttgcatctttgacagatgtacatcaccttctgtttccttcttaaaaaccatgccatgcaatactgaagaggaagtgataccacagcccagaattttacaaactctgatgttatcaactttgaaatggccagaatcaggaaaaatagatacgcatgcctgaacaataagcttggccagaaatacttcattaccatattgtttacacattacagaggtacgaagtagagatgagacttcatcaacatctcgaaggttttttgcagaacaacgtaccaaattaggaagaatctcatgagcttttctgcaagctatttcataaccttctatgacctctgaaactgacaggccaatcctcagaagttcttcagctaattccaggagagctccggcaaataccagaacaatgtttgtgccatctccaacttcttgctcttgcatatgagaagccattacagtcatttttgcagcaggatgctgtacttctagttctcttaaaatagtcgctgcatcatttgtcacaaacaacttctccaagtggttgataaccatttttttcattccatttcgtccatatgctgtacgagtggtttgggcaagctccttgcaagcttgtatgtttctatacacagcctcttctaattctgaaaagtgtttcgctccctccttgagcatctgggcgaagcccggagccttgggaacttgaagcgccatggccagcctgcaggaagccgttcacgtgaccgctcagaagaccgcggaggaaccaaaggttttcatgcctgatgaacctggagatacattcagtcactcttccatctttgctatatagtccagccataccagactacatgcaagtcctggagcataatgtattttttgctgttccaagactttgtctttataattagaatgctatacccttgctctatttgtttggctatctcctattattcaacaaagcctcaatttattttgcaaccaccaaaaacatgcatgctaaaataattaggtgaaaggtttttaggaaacacagtttccaaatgtcaccccactgattaacttcaacgggaaaaaatatctttatagtggagaaacttgatggtatctataccaccttatctaagtggtcaaatttagcattattactgtgagataaactgacataatgtggttcttgatgtgacccactaagatcaacatgtcctatgtagtatatgtgtcaaaaacatttaacctgaatataataaaggaaaaaaattatgcaagtctaaatttagagactctctacaaaacaatgccttgggttcttaaaaagaaagcccatgtcaaagagagaattatttcttatatagaccaatggaacagaacagagccctcagaaataataccacatatctacaactatttgatctttgacaaacctgacaaaaacaagaaatggggaaaggattccctatttaacaaatggtgctgggaaaactggctagccatatgtacaaagctgaaacttgatcccttccttacaccttatacaaaaattaattcaaaatggattaaagacttaaatgttagacctaaaaccataaaaaccctagaagaaaacctaggcaataccattcaggacataggcatgggcaaggacttcatgtctaaaacaccaaaagccatggcaacaaaagccaaaattgacaaatgggatctaattaaactaaagagcttctgcacagcaaaagaaactaccatcaaagtgaacaggcaacctataaaatgggagaaaatttttgcaatctactcatctgacaaagggctaatatccagaatctacaaagaactcatacaaatttacaagaaaaaaacaaacaaccccatcaaaaagtgggtgaaggatatgaacagacacttctcaaaagaagacatttatgcagccaacagacacatgaaaaaatgctcatcatcactggccatcagagaaatgcaaatcaaaaccacaatgagttaccatctcacaccagttagaatggcgatcattaaaaagtcaggaaacaacaggtgctggagaggatgtggagaaataggaacacttttacactgttggtgggactgtaaactagttcaaccattgtggaagacagtgtggcgattcctcaaaaagaactagaaataccatttgacccaaccatcccattactgggtatatacccaaaggattataaatcatgatgctataaagacacatgcacacgtatgtttattgcggcactattcacaatagcaaggacttggaaccaacccaaatgtccaacaatgatagactggattaagaaaatgtggcacatatacaccatggaatactatgcagccataaaaaatgatgagttcatgtcctttgtagagacatggatgaagctagaaaccatcattctcagcaaactatcgcaaggacaaaaaaccaaacactgcatgttctcactcataggtgggaactgaacaatgagaacacttggacacaggaaggggaacatcacacaccagggcctgttgtggggtgggaagagtggggaagcatagcattaggagatatatctgatgtaaatgacaagttaatggatgtaaatgacaagttaatgggtgcagcacaccaacatggcacatatatacatatataacaaacctgcacgttgtgcacatgtaccctagaacttaaagtataataaaaatatatatatataaaaagagagattaaagagacatgacaactaaatgtaatggtgtgattgattacctgacaggatactagatttaaaaagatttttttaaagctataaaaaatactattagggcaactggggatattgccaatgtattaatgtattttatcaatgttaaatttcccacgtgtgataattatatgatggttatgtaggagaatgccctttttcttatacaatatacactgaagtatttaaagtgtcttaatgactgcaacgtactcaaatggtttcagaaaaaaatgtacttgtgtatgtatgctctatatgtatggacctatctacagagatggggaaaggaagcaaatatagcaaacttaacaggtgaatccaggtgaaggatatatgggtgctcattgtacttattattttgcaacttttctgtagatctgaacattttcaaaaataaaaagttggagggaaaataaatttaaaatcagcctctagaaatgttttccctccctggttctctgaggaccccatcctttgtactttcataacactgtatgtatttcttcattataatctgtcctctttcttctcattagagtatttaaggtaagatctattttttgagtctgccatttattatttctgttgccctcgggaaaattacttagtttctctacatctcagtttttatatttgtaaaatgtagatcaaaaattgtggaggccaaagcaactccatcttagaagttaatctaccatattgacttctgatcaaccctggttccgggaatacctctgagatttccagttaatctgttgtttaatagtatgtacttactgtaaatcccacccttagggcaaactcctacccattcgctctgaagtatgtgtgcccctcccctgtggtatatcatccctgggtcaggaggtaatggtatggggatctaccatcttgtctcaccactgcctgagacagacatggcttctgttcataagtccctatgaaatgtttctaagaaactgaatctgtcagcttctttcttcagcctctcagcttcctcagcctttggggtaggtttgcatagacctcctcactgtgaaacaaaaatagtaccaacttatagggctattgtcaggattaagtgagatactgcatgtaactcatttagcactgtgcttatcttatagaaagtcctcagaaaggtgagtgttatttctattactattactattatgtcttctctctgtatttcatgcccatgtatgatgcctggctcataacaggtactcaatgagtaaatgacgcactgtcctcagctatcattttgttgttgggtatcatgcaaaaagaactgatacctgggggaatgagaaaagggttactgccaaagagaattctagattaaaaacccacagaccaatagatcttggacatctgtgggtacaagttagaaatctgatttcagattctatgagtctataggctttcttttcttttcttttctttttttttttttctttttgagacagagtctgttgcccaggctggagtgcagtggtgcaatctcagctcactgcaacctctgcctccagggctcaggtgattctcctgcctcagcctcctgaatagctgggactacagacaggtgccaccacacctggctaattttgtgtttttagtagagatggggtttcaccgtgttggccaggatggtctcaaactcctgagctcaggtgatccacccgcctccgcctcccagagtgctgggattacaggcgtgagccaccatgcccagccactgtgggttttcttaatgtatgggtagaggtggctttactattagccagtgtgaagagtccttattcttgtgctttggccactatccctgcactcccatcctgggaacatacctgtgtttaggcttcaggccaaacatttcatggtcaaacctttggtttatctttttttccaaatatttgtttgctaatgattggccacagatcttccatataaaatgtgtaagtcgagaagagaacaacacatcagcaggatatccgtagtcccctacacgattcaggatccaagcccctctcctggtgctgaggaaaacctggggcatggaagaaattgtttgcttttgtcactcagattcgtaaaccttcaaaagcacccccattttcttcaagaatcatttcaggcccggcgcggtggctcacgcctgtaatcccagcactttgggaggccaaggcgggcggatcacgaggtcaggagatcgagaccatcctggctaacacagtgaaaccccgtctctactgaaaaaccccgtctctactaaaaatacaaaaaattagccaggcgtggttgcaggtgcctgtagtcccagctactcgggaggctgaggcaggagaatggcgtcaacctgggaggcggagcttgcagtgagccaagatcgcaccactgcactccagcctgggcaacagagtgagactccgtctcaaaaaaaaaaaaaaaaagagttcaaactcattagtctggctttttagcccctgcacaatctttgtgggtttttatgtttgtttcctgccattttccttcccaaacactaaacttagaattaaattggtgtatctactgtccaagaatatgttttgctctaatacaccgttgtatttctgtttagtgctattatgcctgcctgaaatgccttctttcctcttaactctgcgaagcctgttcatttttaagacccagatcaagactgcctcctccatgaagaaaccgctgactattcaggctgacaattttctctccatcctctgaatttctctagcacttatcacctgtagaactcattaaaaatcatgtactggtaaagttgaaagcagctggagaccatttaatctaaaaccctcattcttttgccattgacattgttggcattattacaaaaacccctgctatttatcatttttattgatattaaactttctacactcctaatttctgtctcttcaaatgtgttttctcaaggataggagataaagcctacacatccacagcagattatcatcacttccatttattgggatttgtgacctttaagtcattgtgctaggtccttcatctatattacaacaacctcttgaggaaagtattattacacccatgttatagatgaggggcatggaaaggatgaataacttgcctgagatcacagagctagtaagtggcagaggtgaatttccaacccaggtctgactaactccaaagcctgtgcttaagaaatgtttgattgattatttaatggagaaaaataagattgctagtggaacaacaggaagctagtcagtctttctgtgtcctcctctggctaaagttcatgttcagaactgataaagatttgatatgcagttacctggcaaaagaatcacttttcctacactatgaaactctctggagatggcttccagattttaagttatatacgcacattgcttcatagtctttttgtctaaaatgacctgtctacagagggataattgtttacttcacaaatcttatctcgcctaaagtgactgtaagcactctgataattatgtacttccacagtcacagttgaaagagcatatatggtcttagaaactgaacaattttgtgtgctggctatataacttctgctgagtaatgaaaacgctcagagccctaatgaaaagatttcctatttatgaaatagtaataataataatacatatatcacaaggctgttgtgataattaagcagtgtttttgtaaaaggtgtggtatatagtaaacacttgataagtgcttaatggctgtcatatttcttatttcagttttccatctataccttgttttaagcaaataacatttacaaatcagatttataaggaaaattgtttaatcagtgtaatcttatatgaaattaatattgaaaaaaaggaatgttttctctttacaaaagcatctacaagaattatacgaaaaacttccatgatatactgaaatatataggtccatttaaagtttttgatttataaacaaatcatcatgaatacaatttacaagtaaagtaaaaagttagaactcagcaattgagtttcttcagcttggattagtggtgtgacagtattgcctctgctatgcagacatagttttcctttgcattttcccaggctttctcacagacacagccaccttatctgtacccacacagaaatgctttgttatgtggcaacctgcaattccccagagcaggtaaggccaagctcccttagaactgcccatttgacaagccaatgatattaaagatggctctcgccatgggtccccactccacattttgcacattcctctaccataacacccacatacgttttaacccttgtttatataattattttaattatttttaatccttgtttatatgattatttcctgataaatgtctgttgaattaatttatgaagtatcatatgaaataatttttgtggttatagatgaggatagcaatgagaagaagtgtttttcaaacaaagttgctgagtaagagtcatttaacagaattgtagcactaagcttctaattaaaataaaacaatttaaaacatctttatagagaagcatggcttaattaaagttactaaagaacaaccaagacatttacctattgccaatagagtttgattcaacacagacattaataacaaaatacaatattggcatgtctttttccaggaatttatagtgaagacacttgcttctcagttcaaagtctgctatacaaaaaccaaaacaaacaaaacaaaaagccaaggagatataattgctttagaatgaatgttatctgagttacctaactgtatgcaaaggccagggcaagctgcttgcatgtgctacagtttggacgctatacggatacccacattgtctttgggaagataaaattgatacttttttccatttggggagtgtaaaggaaaattcaagcaccatcctatgagtgaaaagtttccaatgatcacgcgtgctttcctttatgtaagaacatagcacttctgctggccaattgaagatcctcgctctcaatactgctttctaacaacctctcccagcaattactttgtctttatcaaagccagaggcacactctgagaagatgcctgattaggataatgagcccagactttagctgatccagttccttggtgtgaggctagttgcacaatggaactctaactggtagccttaactcctctattagcaccaatcaccatgttgccaactgaggtaatgaaacgaagccctatatttgccactggcactgaagggctatgtgcaggtatccctattctctgttgggtccacctgcagcttccttggagaaactgaagctagagttaagcaacgtaaataataattgagtgattcaaacctgcttggctgtttggctaatctctacagccagatcccctccagaattcccaatgccaattataatgactctctttccagtgaatccctctgggttcttatagtctcgactgtggaagtactgccctttgaacttctcaattcctgcaagagaagggaaaataattattgggtaatggtttacatgatagatatcatttgtcaagtcatttgttttttttgcagacttaagtttaagcatatattctccaagtgttctctttactcagctactttcttgcctttctcagtatttttgcctattttcttttcccatagcctcagagtagtaccttgtgatttccttgtcatatgtactttgcttaactcaggatgtgtttgtattttggatttagagatataaatataaactgcctcagaaaacctccattctcttttatcttttcatccccttaaatacctactcgcatttcacttacagcacatatattcttatatactttagagtatagagtgcttttttttttaaaatgaaaatccaggccaaagactgaaattcttcaagctttcattccttccttagaaactcaatatttgtgtttactgctgaaaaattccttattctacctaatgctcctcaagaactccacattcttccctttgatactccagtcatttgatacaatgactaaagtcattgtaaaactaaatagactgcaaattttgctctaatctccaaaattacaaaaatggcagtaatacaagttaccccaacatccttctggggaacaagaataattaggataagtcttacttcattccaaagtaggaattactcagaccacaatcctcccattcctcaggggtcaggtcacaggcatgggtcaagggtcttccttcctggtaagctgctcaccagggaagctttccagaggtagatgagcattggtgtgatggccagtgcaaaccatgactccatcaaagacattcatctcctttttcccttcagattcagtgaccacttcccattggcctgaagtggcaaaatcaggctgcttcttcacactgcacacagtggtctgaaaagaaaagtgataaccacaggggacatccctgacatgactctccttgcatagtgttacacaaagggctgatatcacagacactatcacataataggacccatgcagggatatttgattttcatactccacaaataagaactgtttggggctgtagtcagaatgagaaaatttccacaagacagaaaaaaataacatagtgttggcaggctaatgtaccctcctcttctagaaaagtgcaagtcaccaggtctcttggtccaggtcctaaggcactgtaacacctgagtaaagcctgggcttctcctgtgcttttatgacactccatgcactaaatgcctattcttctcctgacccctatatgtcctgagaccttctgatgtcttcttaccctaggttctcttctcctggctacctttaaataagtgactgagctatagggctccttttcctggtagggtagaaaaacacctcagtggctctcattttatataaatgaatctccctttggctcccataaatacccattttacaaagaactataaagaaagaggctgtgaaacaggatagtgttatgatttttagctttataaaaaataataaatatgggttaccctacttaggttaaggaaacactatgtgcttctacgggcccatgaccataatgtcttcatggactaatagagacaccatcccggccgggtgcggtggctcacgcatgtaatcccagcactttgggaggctgagccaggtgaatcacccgaggtcaggagttcaaaactcacctggccaacatggcgaaaccccgtctctactacaaatacaaaaattagtgggtgtggtggcacatgcttgtaatcccagctactcgggaggctgaggcgggagaattgcttgaacttgggaggtggaggttgcagtgagccgagatcgtgtcactgtactccagcctgggcaacagagcaagactctgtctgaaaaaaaacaaaaaacaaaaaaaaaaagagagacaaaccacccctgcatgcactagcaatccagcactatttatagttcctctatcatgttcttttacacaggctggtgcctctgccgagatcacccttttattccttatttggtagactcctactcatccttcaagactcagctttaagaaaactttatcttctttaagaaaacttccctggaacctgatatttcatgtcctgatgggttcaacatctttcctccgagctgcaacgtatagatctctagcatttgtccccatgtaactctctatttttattaattatatttataataaaatttttcttcatttttatccccttaactagactataaagttactgatttttcttttttgtctttgcatattcaatgcttagtatggtagcaaacttgttcaataagtattgtttaaataaatgaagagaagcaccactggaatgtaaatgacttactttagaagttcactagatgttttcattttcttattgtcattaagcagaaaaaggcatgacttagcaggatgatcagaaggcagaaggtttgggctttttgccagctgtcagaaatatctgaccataaaattcttttatggtcatgatcagaaattatagaaaagtcctagaatactttagagcaggaaggaaccacagaagtgatctggtacaatcatcttgttttacaaacaagaaaatttttaaaaattgaaattgaggaaattgcttgtctaacatctaagttagttagtggtagggcaagcaccagaattcaggtttttattctgcaattccatgttctcccctctacaccagagttaactacccaagagctatactttactgggtttttatgatgttcatgtaaacaaatatattggaaagtacttcagaaagtacaaaagggctaagcagtaatggacaagttgtggaaccagagagttttaaagttcccatacctatcagttcccttctgtaatggggaaaacatttcccttcatctgtttattgcaatcaaataatgtgaaatgaaggtaatgaaaacactctgccagctggcttcctgtatctgcagccaaaatatatgaaagagagactgtcccttgaatatttttgaggagcaaaggaggacaaagaatggagtttttgcctgggtaggataaatacatgtgcaaatcaagccaatctttagaagtaaacattggtaactgaaaccacgttattcatttacttggcaaacaacttcaaacacaaagatacccacacaattttctaccttaaatcgaatatactttagaaggtcaaattctttggcatacatcctgaaatactccaggacctgggcattatgcatgaagttgggataatgatctgggattggatagtcactgaagcacatcatctctttagaagtattgatgatcactgatttgtaaatactggcccttccttcttcaggattttcctgcaataaatagaaagtattcatagcaacttgaggatcatcttcatgttttataatagccaatagacatctgaaaaagttttctgaaagaagtgtcaattaaatcacacacacaccttccagtatttgtgcccttatgtagtcccttccccttgaatctcagttatctttatgacttgcttttgaccaacagcatacagttgaaatgacactgaatggcttccaagaccaagtcataagtagccttgcggattctgcctgggtctcagaaagctcgctctggtagaagctagcagccatatgagaaatccaactaccatgagaccaccatagcttgaggaagtccagcctcaccacatgaagagaatgtctgggacagaaaatatatggccagtccccaaaaattctacctattctattctatcccagctgaagttctaaacatgtgaacagaaagttactaacactgagtaatagtcttttaaatgagtaacaatgaggcaaaatgggaagatacacaggaaagagtgtaacagtttccatatactggaaagagtataacatctccagcgttttctggagagcagtgttaaaatgtatatgaaactccttgcaatttacctagccttttaaaaaaatattcagcatcgcttaggaagatttatgttaaaggatgttaataccagcattattcataatacaaaaatgagacaagctaaatgcccaaaaaaacaactgaaatttgagaaccactgctctagatccttactaccaaagtatggtctgtagactagcagctggggcttcccttgagagattgtgttagaaatgcagactctcaggccccacctcagacctactgaatcagaacctgcatcttagcaaaatcttcatgtgattcagaattcagatgctcatgcaaactgagatgcactgcattaaatgacattaatcctcaattcagtgttctttcccctacaacaaacttctttgcatcctcaaaaacttcctattgaggccgggcgtggtggctcatgcctgtaatcccagcactttgggaggctgaggtgggtagatcatctgaggtcgggagttcaagaccagcctgaccaacatggagaaaccctgtctctactaaaaatacaaaattagccgggcgtggtggcgcatgcctgtaatcccagctagtcggggggctgaggcaggagaatcgcttgaacccgggaggcggaggttgcggtgacagagatagcgccattgcactccagcctgggcaacaagagcaaaactccgtctacaaaaaaaagaaaaagaaaaagaaaaaaaaacttcctattaactatcttatagcattgttgtggtgatcacataaagtaatgcaatgatgcaatctacccagcctgtcaccgagatttcacaaatgaggagttttcaaatttttagattttcaaaaattgttttgactatggaaaatcaccttaatcaatttggatctcctcctccctttttattctagaaatgaacagatattgagatattgagtattatgaaacattaaatagccacaaaggagagtgtttgttgtttgttggctttgtccacctttaggattgtttttctcccatttttattgcttaattattcaatctaggaatcctaaattgatcattcccatttctctgacctataatccaacatctcatttctttaactgctaataacattttcataagactcctttgaagtctcttcttctaatctagcctacctgtttcaaccaaagtgttctctctaaggtgtggctggactaaatctctgccctaattaaaattttagatgttttcccatttcctgcagaataaagttcctatttctcagcttaggattcaaagacctccataatgttttgtagtgtattccttatctctccaactagattgtaagccccttgaattgtactcatggttttccccacagcatccacaatgataaatagcactcaataaatgtttaatggatgcatatcaaattgtattgagaaagggatatacagaataagatgtaagtttcacaaaatgcataagaaaactaataaaatacatcaacatttatctcaaaaagacttcaataagatatatgtatctcccaaaattttgtcccaagaaaaatttcaaaataatataaagtcaaatgcatagatatatttttgtataacttaaatagcaattaattagtaacaatgttaaatgttcccaaaatagatgaatggtttagtaaattatagtatctcaacatgcagaatttttttttttgagatggagtctcactctgtcgccaggctggagtgcagtagcacgatctcagctccctgcaacctctgcctcctgggttcaagcaattttcctgcctcagcctcccgagtagctgggcctacaggcacgcgccactatgcctggctaattttttttgtgtttttagtagagacgggtttcaccatgttagccaggctggactcgatctcctgacctcgtgatccgcccgcctcagcctcccaaagtgctgggattacaggcgtgagccaccgcgcccagcctcaacatgcagaatttaccttccacaccactccatgggtatcctgataaatacaaagtagatcctgccactccactgcttaatagtttctcttgattccatatggaaaacaaaattccttattttgaaatttagcacatttcacaatctagcccggtttatcttttaatcttcatccagtgttgtccttatttaatctcaaatttctaagttattaaattgttcctgaaacactctaggctcttgcacaactttaaaccttcgtaaatattactatttcttcatctggaaaatttcctgtccttcaagagttacatcaaatgtcacttccttcaacaagacttttctaatttctccagagaattagattccgctattcatcctccaagctcccaaaactctctgttcatatttctataaagataacttaaacacactatattatcaggcatttgtttccatgactgtgagaaacccgagagtagccatatccttctttaaatctctattatcaggacctggtgtgtactggatgtgcaataaatgctttgaaatgaattagttaatgaattatggaaattgaatttggagacaccaaaaactatgattttgaagtctgtgcaggaacattaaaaatggcgtatgatataatgaagtacaaagggaactgtaaaattaaatttacattctaatcaccaaatatgtaatattatgtctatctatgggtatataattatacttgtataatcgctccctgttagacatgtctcttttgagtatacttcatttatttgaaatagaaaaaaatgtgaaaatacagaaaaccagtcgacttattaaggcagtaggattgctttctttttcttttatttttgttaaaatgttgtttgtacaacacccattcatgatgaaaactctcagcaaactaggaatggagagaaacttcctcaatttgataaagaacatctacaaaatacctataaccaacatcatacttaacagtgagaaattagacacttttcccctaagactgggaacaaggtaaggatgtcctctctcaccactcctatggaacattgcactagaagtcttagctagtacaataatagaagaaagaaaagtaaaggatattcggattgggaaggaataaagataactttttatttgcagatgacctgaccgtctatgtagaaaatcccaaaggattaaaaaaaaaaagtaagaaaaaaagaaaaaaactcctagagtcaacaagtgagtacagcagggttgcaggatacatggttaacatacaaatgttaattgcttttttttttttttttgagacagagtctcgctctattgcccaggctagagtgcagtggcacaatctcggctcaccacaacccctgcctcccgggtgcaagcaattctcctgcctcagcctccggagtaactgggactacaggcgcatgccaccctgcccagctaattttttgtatttttagtagagatggggtttcactatgttggccaggctggtctcgatctcctgacctcgtgatccacccacctcggcctcccaaagtgctgggattacaggcatgagccatcgcacccagtcatttgcttttttatatactagaatgaacaactggaatttgaaattttaaaaactccatctatagtaatacccctgaaattacatacgtaggtataaacataacaaaatatgtataggatttataagcatgaattagaaaacacagatgaagaaagtctaagatttaaataaatggagagatattctgattcatagactagaagattaaatattgttaagatgtcagttctttccaacttgacctatagatacaatgcaatctcaatcaacatcccagcaagctattttagaatccaagctaacacatggattctaaagttcatatggaaagacagaaggcctagaatagaagactttgtccttaatagtgggctgtgcatagtgactttgttccaaagagtatagtatggcaatggagaaaaaaggagcaactttacagtgtggcaaaaactgacaaacgctatttcaagccaggacatcaaggttaacatcaatagtgatattatctagggtttttatagttttagattttacatttaactttttaacgcatgttgagttgattttcatatatggcaaaaggaagggatccagtgtcaatcttctgcatatggctagcagttataccagccccatacaatttatccttgtaacaaactttcatatgtacccccgaacctaaaataaaagttggaaaatgaaaaatagaaaagtggaacaaacttacacttcaacaaagatatattgtggcatatattgaatgctaatttcttacttataataacataaaatgagttttaagtttccaaaaaaaaaaaaaaacagtgggtataatgtggatagtatgtacccttgatgggaggtgaggagaatggcaccttataatattcctccccaaaagtcataaccccaatttaaccatgagaaaaaaataagataaatcccaactgagggatattctacagcatacctggccccaaaactatcaagggcatcaaaaacaaggaaagtctaagaaatttcatagccaaaaagagcctaaggagatatgactattaaatgtaatgcagtatcctggatgggatcctggaacagcaaaaggccattaggaaaaactgagtaaatctgaataaagtatggacttcagttaataataatgtatcaatattggttcattcattatttaaaaacgtatcatactaatgtaaaatggggtaactggacatgaggtgtactgtaattctctgtattatcttcctaataaattttgtaagtctaaaactgttctaaaattaaaagcttatttaaacatgtttgtacataagtgtatatattttttaattaaggtaaattaatgaatggcaaggtcattttggaattaagatgtttgctgtatggagagcaggtgaggcatgttcctaacttctgaatttcatttcatttattcattcaagagatatttagaaagtccctctgtaataaaatactttatgaggtactgataaatgcaagtctgtatgtgtattccaaaagttcaacgtttacaaagagtagagccatcctatccacagcaggtctgttgggatcactgagtgaaatgaatgacagatctcacctctttgaggtactcctatatttcaactctttttcaaatcactaaccacaacaagtgttatcctgtgtcaacaacatccttcaaatccttcgaaacacctgattggaacttaggtaaggtttaccactgtgccaatccactgctttccaaaagagtgagcacagagcagtattgggttagtgagtagaagaaaaagaagcttctgctcctgcattttacaattttctaccattgatgaataaatcttctctctacaaactctatacactgattatatttcctacctaggcacaaggctcacacatttgagcaggaagtctgtgtaagaaaagagaggctaggcacggtggctcatgcctgtaatccccacaccttgggaggccgaggtgagcagatcacttgaggtgaggagttcgagaatagcctggccaacatggtgaaaccccatctttactaaaaatacaagaattagcaaggcgtagtagtgcgtgtataatttcagctacttgagaggctaaggcatgagaatcacttgaacccaggaggcagaggttgcagtgagctgagatcacgccactatactccagcctgggtaacagagtgagactctgcctaaaaagaaaagagagagagagcaggggatggaagttggggaaattggaactgatgggattggaagaagtaataaggacagaagaaaggagaaaaatttaaatgggaggaatgaggacagtttggggcttctgttcctgtcagattttcaaaatcccatggaatagaaactctctttgaactgttgtctgcacattggaatcatctggggagctttaaaaaatggagatagtagaatacatgcttggctctagaaatataacggtgaaccacacaggtgtggtctgttggaacagaagtcagagcgttatgatgaaacacagcttatttattttcaaggaagcagtttacaaagtgttaaaattttgccaagtggataatcagaagaaaaacctccacgttaagtctttagcagagaataagtttaaaccacattggagataaaaaccagaaacttgataatcagacaagatgatggatgccctcccaacctcctcccatcctcaattgatttcatgccttttcagtaactgccaaaactggctaagatgcttagtaaagacaccacatgtgtgagtcccatcctaggcctactgaataataaccaacatgtaacactatgttcctggcactgttgtaagtgattggcataattatccattcacttactcctgacaataactctataaagtggatactattattatccacttcttaaagatgaagaaacacaggtacagagaagcttaatgatgtgcccaaagtcacactgctagtaggtgacagaaataaggtttgagcctaagactgcattcttaacctccataccatattgtggctggattttaagagcagaattttctgctgtttactaaaaacaacaggcttttagcccatgtccaagactgatgatgatacacgtatgcaggtcagctaaggggatccactccagatctgaataaggatgattgtcacataaaattagtccccaaaacagagtcagggtgcaaaaggattgtatttcggttcaactaagaaatgctataaagccacttttatgtagctggccaacaatgtgttagtttttatgaaatatgaaacgtaaaacttatctagggcacctcaatactattaaatgttcagaaaactagcttaaaagcaaacccgttctcctctagccacccaagatgccaataggaaagaaggctaagggaaagaaggcggcccccgcccctgctatcagtgaagaagcaggaagacaaaaaagttgtgaatcctctgtttgagaaaaagcctaagaattttggcattggacaggacatacagccccaaagagacctcaccctctttgtcagatggcccccctatatcaggttgcagcagcaaagagctatccttttataagctgctgaaagcacttcctgccattaaccagttcacccaggcttcgcactgccaaacagctactgactgcttacgcgggcccacaagcacagaccagagacaaaacaagagaagaagcagagactgttgtcctggactgagaagaaagctgctagcaaaggggatacccccatcgagacaccacccgtctttccagcaggggttaacacaatcaccaccttggtggagaacaagaagactcagctggtggtgattgcacacgatgcggatcccatcgagctggttgtcttcctgcctgccctgtgtcccaaaatgggggtcccttactgcattatcaagggtgaggtaagattgggatgtctagtccacaggaagacctgcacgacgttgccttcacacaggttcactaggaagacaaaggaggtgtggctaagttggtggcagttttcagaaccaattacatggacagatatgatgagattcgctgccaatggggaggcaatgtcctgggtcctaaatctgtgggtttgaatcaccaaagtggaaaagggaaaggtgaaagaagttgccactaaactgggttaaatgtacactgctgaattttctgtaaataaaaagaataaaaattctccttcaaaaaatgtaaaaataaaagcaaacccagcaaatccaatgcatgtcagtttggagatcaataaaggtggctggtattctttggaatataataagtttaactatctttttttaatttttttccttgagacggagtcttgctctgtcacccaggctggagtgcagtggggcgatctcggctcactgcaagctctgcctcccaagttcaccccatcctcctgccttagcctcccgagtagctgggactacatgcacccgccaccacgcccggctaatttttttgcatttttagtagagacgaggtttcaccgtgttagccaggatggtctcgatcgcctgacctcgtgatccgcccgcctcggcctcccaaagtgctaggattacaggcgtgtgccaaccgcgcccggccacctgacactgttaagataaactgtcgtatgcacctagttgcagggagggtttcaagtattaagggactaggagatgtatgtacctggaacctccagagccctccgatgtcatcagtcctttcaaagcagacaggttccaagccttcttctacgcagcacttgatggaagagagcccgctcactcctcccccaatcacagcaattcttttcttagtcatggtctcccgagatcttcacctgttagtgtcgcctgtcctaaagaaaggatgacaaaagacaaaaagcacacatcggttaacatttttcaaggaagaccttggccgtggcattcgaataaattctgtacaagaggtgtcttgaggaggacagattcgacggtcctcttcaccagaggaaatctttctgctggcatgggggagccctgcgcctgcaagacccagagctgagagtgctctgctgcggtaccggatctcaccgcctttcctgaagcgctcaacagatccttcagctgcgatctggaggagactcaacaggcggctgttgtcaaattactataaaccaacaacggacaaacagcgagagccaacggggaggggctgtagcactccacctcctttcagggaccactcccccgcccactcagcggcacccattctccctccctcgatgggaataaaacgtgggctgaagctgctttgggcgaaaaagttaatcctacaacttctctatatttcagctgctgttgccagcactctcaattactttctctgaaacccctagccccgtctgtgctcgcttctgcatccacttttaacttcctggtttttgccttaaagtgacaaacacttcctagtgaagggaaaactgtcaacaaccccaaagccagttctactccaaatgcttaaatgaacacctacctttcaggtgatctgttcaaacagattgtagcaggatgagccacagacaaaactcctcagacaccgaattaaagaaggaagaggtttttattcggccgggagcgtcggcagactcgcgtcttaagagccgagctccccgaaaaagaaatttttggcctttttaaaggcttacaactttaaggggtccacgtgaaagggtcgtgatacatcaaacaagagtgggaaacgtgactgggggctacaatgcttttttcatacagtgtcaggaattcacagataacacaagtagtttaggtcaggggttgatgttattattattactttttttaactcctagggccgggtggtggtgccaaggttgtctggcaatttatcttacttttttttttttccaactttttgctttttctctcctcctgtcttgtgaacgaggcaaggtggtgggaggagggcagcagtagtagcagtggtctccttccttaagatgatcctgcccccacttccgcccccggctcacctatacctctctcctcccctcctcacaatctggatctaagaatctacacttctggaagaaatttacttttaaatccccatgcactgagctgagtgctggagtatagtgaggaatgtattgtttcctactcagaggggcttacagattagtggaggagaccaaaacataaacaggtaattttaacgaaataaaagtatttttaatagtgctttcacacagttatattagtaaccaaaaatacaaaatatccacttctaaaatgtaacttttcaaatataaagtcatgtagaaccaccaatataacagatacaagatttcaggcactgggttagaacaagggcccatccagacaagggttctatttgacagatgtgaggggttgtaagaggcatggattgtggctcatgccttggatccttgctctccttctaccactccctgagtcaattttgctcttccaatctgcacctgctaatcttggactttttcatgagaggcaactgatattttgtttgtgccattgaattttttgttgtatttatagcaacttagcagactctaattaacattaatgtgttttggaactgtcgaacttttttttttttgaaacagggtctcactctggcacttgggctggagtgcagtggtgcaatcatggctcactgcagcctctatctcctgggctcaatctaccctcccacctcagccttctgagtagggactacagctgtgtgccaccacacctggtaatttttgtattttttgtagaaatgaggtttcactatgttgctcaagctggtcttgaactcctgggctcaagtgatccacctgccttggcctcccaaagtgctgggattacaggcatgagccaacaaggccagcctgtaaaatattttaaagactaatatctttcacaaaagcattcaactataaatgtgaatttatactaaaatagtatcttttaaaaataaaattctgaagacagtgtttcaacacaaccattttatatgctagaagttaacttaaaatgaattacttgtaaattggataattttgaatgcactagaagaaatgcctaaaggaaaacatgaatacttttataaactgagtattaatttcctcctactgaatcagttttacaaataatgcaagaattacttttaaaatgtagttaacaatgtaattttattttaatgtccccctacttcaattgtgtcttataattaattgcttttgaatatagcaaatatgttttgtgttgtattaaaattacttatacaatgttttaaaccttgactcaaatgttctctctcttgcctagctgacaatttgcaagtaagtcaatttcttcattgaaaaataacttgatacatccaaattaatatacagactcaactcagttactcatgctattactagacagcaatattatgagtgagaaataagaacaactaattccaagataacatatgaggcttttgaaggagtgtatgtgtatggatgcacatgcatgtggaactgggtttgcagagtttctgcaaaggtccaacccagaaagagctttcaaacaatacagtctcacctctactcagatgctaccctgttttctaattctttctattacgtttgcattttgcccatattcattcagcaaacagtctcttttggaggccccctttgttttgagatggagcctcactctgtcgcccaggctggagtgcaagtggtgcgatcttggctcactgcaagctccatggaggccacttttttttttttatcatactttaagttttagggtacatgtgcacaacgtgcaggttagttacatatgcatacatgtgccatgttggtgtgcagcacccattaactcatcatttaatattaggtatatctcctaatgctatcccttccccagccccccaccccacaacaggccccagtgtgtcatgttccccttcctgtctccatgtgttctcattgttcaattcccacctatgactgagaacatgcggtgtttggttttttgtccttgcaacagtttgctgagaatgatggtttccagctttatccatgtccctacaaaggacatgaactcatcattttttatggctacatagtattccatggtgtatatgtgccacattttcttaatccagtctatcattgttggacatttggcttggtttcaagtctttgctactgtgaatactaccacaataaacttacatgtgtatatgtcttcatagcagcatgatttataatcctttgggtatatacccagtaatgggatggttgggtcaaatggtatttctagttctagatccctgaggaatcgccacactgacttccacaatggttgaactagtttacagtcccaccaacagtgtaaaagtgttcctatttctccacatcctctccagcacctgttgtttcctgactttttaatgatccccattctaactggtgtgagatggtatctcattgtggttttgatttgtatttctctggtggccagtgatgatgagcattttttcatgtgtttttggctgcataaacatcttcttttgagaagtgtctcttcatttcctttgcccactttttgatggggttgtttgtttttttcttgtaaatttgtttgagttcattgtagattctggatattagccctttgtcagatgagtagattgcaaaaattttctcccattcggtaggttgcctgttcactctgatggtagtttcttttgctgtgcagaagctccttagtgtaattagatcccatttgccaattttggcttttgttgccattgcttttggtgttttagacatgaagtccttgcccatgactatgtcctgaatggtattgcctaggttttcttctagggtttttatggttttaggtctaacatgtaagtctttaatccatcttgaattaattttttataaggtgtaaggaagggatccagtttcagctttctacatacagctagcccgttttcccagcaccatttattaaatagggaatcctttccctatttcttgtttttgtgaggtttgtcaaagatcagatggttgtagatatgcggcattatttctgagggctctgttctgttccattgatctatatctctgttttggtaccagtaccatgctgttttggttactgtagccttgtagtatagtttgaagtcaggtagcgtgatgcctccggctttgttcttttggcttaggattgacttggcgatgcgggctcttttttggttccatatgaactttaaagtagttttttccagttctgtgaagaaagtcattggttgcttgatggggatggcatttaatctataaattaccttgggcagtatggccattttcatgatattgattcttcctacccatgagcatggaatgttcttccatttctttgtatcctcttttatttcattgagcagtggtttgtagttctccttgaggaggtacttcacatcccttgtaagttggattcctaggtattttattctctttgaagcaattgtgaatgggagttcactcatgatttggctctctgtttgtctgttattggtgtataagaatgcttgtgatttttgtgcattgattttgtatcctgagactttgctgaagttgctcatcagtttaaggagattttgggctgagacaatggggttttctagatatacaatcatgtcttctgccaacagggacaatttgacttcctcttttcctaattgaataccctttatttccttctcctgcctcattgccctggccagaacttccaacaatatgttgaataggagtggtgagagagggcatccctgtcttgtgccagttttcaaagggaatgcttccagtttttgcccattcagtgcgatattggctgtggttttgtcataaatagctcttattattttgagatatgtcccatcagtacttaatttattgagagtttttagcatgaagggctgttgatgtgtcaaaggccttttctgcatctattgagataatcatgtggtttttgtctttggttctgtttgtatgctggattacattaattgatttgcatatgttgaaccagccttgcatcccagggataaagcccacttgatcatggtggataagctttttgatgtgctgctggattcagtttgccagtattttattgaggatttttgtgtcgatgttcatgagggctattggtctagaattctctttttttcttgtgtctctgccaggctttgggtatcaggatgatcctggactcataaaatgagttagggaggattccttctgtttctattgattggaatagtttcagaaggaatggtcccagctcctccttgtacctctggtagaattcggctgtgaatccatctggtcctggactttttttggttggtaagctattaattattgcctcaatttcagagcctgttatcggtctattcagagattcaacttcttcccggtttagtcttgggagggtgtatgtgttgaggaatttatccatttcttctagattttctagtttatttgtgtagaggtgtttatagtattctctgatggtagtttgtatttctgtgggattggtggtgatatcccctttatcatttttattgcatctatttgattcttctcttttcttctttattagtcttgctagcagtctatcaattttgtttatcttttcaaaaaaaaagctcctggattcattgattttttgaagggttttttgtgtctctatttccttcagttctgctctgattttggttatttcttgccttctgctagcttttgaatgtgttcgctcttgcttctctagttcttttaattgtgacgttagggtgtcaattttagatctttcctgctttctcttgtgggcatttagtgctataaatttccctctacacactgctttcagtgtgtcccagagattctggtacactgtgtctttgttctcgttggtttcaaagaacctctttatctctaccttcatttcgttatgtacccagtagtcactcaggaacaggttgttcagtttccatgtagtggagcggttttgagtgagttccttaatcctgagttctagtttgattgcactgtggtctgagagacagtttgttataatttctgttcttttacatttgctgaggagtgctttgcttccaactatgtgatcaattttggaataggtgtggtgtggtgctgaaaagaatgtatattctgttgatttggggtggagagttctgtagatgtgtattaagtccacctggtgcagagctgagttcaattcctgtatatccttgttaattttgtgtcacattgatctgtctaatgttgacagtggggtgttaaagtctcccattattattgtgtgggagctaagtctctttgtaggtctctaaggacttgctttatgaatctgggtgctcctgtatcagtgagactctgtgggtgtaggaccctcggagccaggcatgggatataatctcctggtgtgccgttcgctaagaccattggaaaagcgcagtattagggtgggagtgacccaattttccaggtgctgtctgtcgcccctttctttgactagcaaagggaattccctgacctcctgtgcttcccgggtgaggcgatgcctcgccctgcttcagttcatggtcagtgcactgcacccactgtcctgcacccactttctgacactccccagtgagatgaacccagtacctcagttggaaatgcaaaaatcacctgtcttctgcttcgctcatgctgggagctgtaaactagagctgttcctattcagccatcttggctccaccccccagaggccacttttaaatggcatctttgtaagatagaataggcttgaatcttgagggagggctgcaaaggaaaggtggctgacaagcattggactgtgacatgagtgagaaatatactttttgctgaattaaaatgtggagagctatttgttcagtagtaaaccttaataagtcaatcctgactagtccaagagtcatttctagcacagtgtctgttgggaaaaagctgagtgttgggaagaaagctgaggcagggcttgcatgtctgacataatgtcctctggaatgtgtgtagacttgctggatccttgcttctagccctccaagctcctagagcggttgtattcccattatctcaagtagcagaacatgttccatataaatgctaaacctcaacctctccctctccctctccctctccccatggtctccctctccctctctttccatggtctccctgtgatgccgagccgaagctggactgtactgctgccatcttggctcactgcaacctccctgcctgattctcctgcctcagcctgccgagtgcctgcgattgcaggcacgcgccgccacgcctgactggttttcgtatttttttggtggagatggggtttcgctgtgttggccgggctggtctccagctcctaaccgtgagtgatatgccagcctcggcctctggaggtgccgggattgcagatggtgtctggttcactcagtgctcaatggtgcccaggctggagtgcagtggcgtgatctcggctcgctacaacctccacctcccagccgcctgccttggcctcccaaagtgccgaaagtgcagcctctgcctggccgccaccccatctgggaagtgaggagcatctctgcctggccacccatcgtctgggacatgaggagcccctctgcctggctgcccagtctggaaagtgaggagcgcctcttcccggccgccatcccatctaggaagtgaggagcgtctctgcccggccgcccatcgtctgagatgtggggagtgcctctgccccgccgccccatctgggatgtgaggagcgcctctgcccggctgcgaccccgtctgggaggtgaagaacgtctctgcccagccgccccgtctgagaagtgaggagaccctccgcctggcaactgccccatctgagaagtgaggagcccctccgcccggcagccgccccgtctgggaagtgaggagcgtctccgcccagcagccaccccatccaggagggaggtggggatcagcccctgccaggccagccgccccgtccgggagggaggtggggggtcagccccccgcccggccagccgccccgtccgggagggaggtggggggtcagcccccccgcccggccagccgccccgtccgggagggaggtggggggggtcagccccccgcccggccagccgccccatccgggaggtgaggggcgcctctgcccggccgcccctactgggaagtgagaagcccctctgcccggccaccaccccgtctgggaggtgcacccaacatgctcattgagaacaggccatgatgacaatggcggttgtggaatagaaaggggggaaaggtggggaaaagattgagaaatcggatggttgccgtgtctgtgtagaaagaagtagacatgggagacttttcattttgttctgtactaagaaaaattcttctgccttgggatcctgttgatctgtgaccttacccccaaccctgtgctctctgaaacatgtgctgtgtccactcagggttaaatgggttaagggcggtgcaagatgtgctttgttaaacagaagcttgaaggcagcatgctcgttaagagtcatcaccactccctaatctcaagtacccagggacacaaacactgcggaaggcggcagggccctctgcctaggaaaaccagagacctttgttcacttgtttatctgctgaccttccctctactattgtcctatgaccctgccaaatccccctctgcgagaaacacccaagaatgatcaataaaaaaaataaataaataaatgctaaaccgtcacagctgtagatcatgagcctgctcttttgacccccacattctcaccacctgattctctgttggattaccaataaacagcgtgggctcccagagctcggagccttcgcagcctccacaattgtgatggccccctgctcccactttacttctcaaactgtggttttctcaatcctttgactctaccggactttgtcacccccaggatctggtgttgggtctgatcaccccaacagcatccattctatgcctgctatgtgctaggtactttgttacccagagaggaggaagagaaagtgcatatctaaaaaagatgaggagataaatcacagccatcatggtaggctgaaaacatcgtccccaaagacatccatgtcctaagccgcagaacctgtggatgttataacacatgtaaagtgcccacacgtggcctggcatgtagttggagttcaagtattagtcagcattaattgtaaaaaattattttgttttctaacttaaaaatgtttttactaatttattttgaatggacaaataacaattgtctatatttatggagtaatagtgaaaaatttgaaatgacttcataaacgttcatcaagatggggaaggactatattacatattatatttaatgagatgaatttatactgacatgaaaaaattatgaaagattttaaccagcatggcccttatttcatttgtatagtttccatggcagagggtaggaataatttgggcaagcacatttaaagcttcaacttatatactagggtaaatcacatccactcatattccactgtccaaggcaaatcacaggggttcttcctattaggaagcactgcaagtcacatgactaagggcataaatgtataaccatcttgtggggagaaagtggatagttaggaacagtaatacaatctatcaaagctggttagagcccaccatggagtagatatcccacactgtgtgtgtgtgtgtgtgtgtgtgtgtgtgtgtgtatgtgtgtgtgtatttctgtttacttttatgacccatatctgtgggccacacatatggggaaaacactatgcctgtagacaccccaagcaaatgagattaccatggaacctcaataatgagggataacttccaatttcttaattctccactgatgagatgtggatacttgagtgatccccaggctcattcccaagtgaagattttcagtccttcgtaataccttggacattcaaatttgtatttagtttcttgtgaaaaaattttcatttaatttttacaacagcattataggatagctactattatcctcataattcactatgcattatgggcctttcagaagcactctgattgttaaaaccctctaattaggaagcctaattagacatgccatttttgagcaatttgaggggatagaggtggggaacccccttgcatcaaagttataactgtgcctcagggatagatacatgtgcaacagaacccagaataggtatgctcatttttcaaaactaaaacccaggctttatagggttagggtaaaaaaaatggctttggattcttgtcaatcagaggaagaagaaggtcatagagagttcttagggtcataattttacattgcctaaaaatattttagagtagggtgaatcatgagaaacattttggcttcctatggtatattattgagacaacctgtcccctacatggaaatattgtcacgggattcttggggtgttgctttgtgagacagaaacctctgtggccattggtacttttgcacaagttttgctcaagcctattgggcttgtttggtccattcagcctggcaggctgcacatggctcatgctaccagcctggatcccatgccagccaagggccagccagatgcagagcagagaggggtgtgtgagcaaatatgaggtccagccactatgcacagccaggcatgccagctgtggcaaggcaggcagctccaggtgccagtatgggcactgactccctgtgaggctccagctggaccaggggtgccacaagcagatttcatggctggcactggagaatgcagtggtgcctggaagcttggagatgccaagagctaaagagccccaaagagggtgtcacagccctggctcagtgagctcctaggtctgggcttcccaaagggctgcagctcctctctccttctctcttctctccttcttgttgcccacaatgtggcaagcaatgggcatgtttcagccctgtttgtgttacaactcttttagctccaccatttggcgggtcctgagttcttgtcctgcgtccaagtagaatgatgtaagttgacaagtggagggtaagcaaggtgaagagaaactttattgagtgacagaacagctcagaggagacccacattggatagttcctctccacaggcaggttgtcccattgagtgttcagttctcagcagagaggagaccctggagtgggtagctcctctctgcagttggttgtcccaatgtctgcttagctctcacagagaggagaccctggagtaagcagctcctctccacagctggcaggtcatcattgtcaactcagctcttagcagagagtagaccctggggtgggtagctcctctctgcggctggttatcccactgtctcaagtctggctgagtctggggcttttacaggcctcagaggagaggaagtgtgcgccaactggtccataggcacccagataaaacacaagttctcactctggtttttgggaccagcagcccagcctccaggcttcaggccctccccagcttgagggtaggtcttcaccggtgacctgctcccttccacccaggagactgcctcctgctggcattcacagcacccaaactgtttgtgcaaaggggcacctgcaggcaagcacagaggctgagctgccccagcacccccttggcctccctcccatgctggcacccaaagtcctgagggggccaaagccatgtgtcagtgctgcctggagtgggtgcacacctggccaggctgcaatagcacccagcctcagctccaaccttgctctgggaatggagtgggtgctgggagcagaaagaggccaggcaatgggaggagacacttcttagcctgcaggaatggggtgggaggtcttacagggcccccaagagtgcagagatgcccaggtctgcagctgtggtttgagcagctatagctgcacccaggagggtggggctcctgcctgctccaggaacccaagagcacagggaggccgagttggtggacatgactcaggcagctgcagctgtgcctgagagggtagggctcctgcctgcttttagccccaaagagcacagggatgcccaggtctgcagctgcagctgggcagccacagctgtacctggggagcaggaagctcctgccctgccaactcagaaggaggcagggcctccacctgttcctggttcccccagctccatggagctggcagccctggtgtgccacccccattgcaagtggcatcatgacagcagctgctctagataggccgtcactgccatcaatatgtcacaaaagttaaatttccagtttggcaaactcaaaagccttcagggactagctgggcagattgcataaacgttacactgctggttggagaacataaagaatgaaattctgggtgaccaatgtgatggcatggcatgacagtcaaaaggcatccagttaaaaaggaaaacactgtcctttcaagcaaaaagaccgtgggcaaattttgatgcctacaatttctaaactatgttctcaaagattaacttgataatattactattttacaaccttacctttgatagtaaaagggagtggcaattctctgaggtgactgggcaagagtcctgtgaaaccaacttactttttttctatacttctatactgtggtatattttccctggctttctgggttctaaatttattacatgttatttcatgacaaagaggtatactggcatcaaaagtcaaaacacagtttttcatttcttgcaagaaagaaaacccaagttaagtgtttttcatcccagcacaaaaatcttccacccatgggcacggacctaattctaacctaagctcaaagttccaagttcatttactcaagaggtctgaataaatgtttactttggtcacagcttttatccaatttccgtatctgactcactaggtgcttctaactggtgccctgatgttacctaacagagcaaggatacaacaaacagcaaacataatttgtttcttaatctgtgcttaatccatgcttgttttggtaatgtctgcacatgctaagtcccactgacagtgttagttggttagcattaatcttatggagttgctgttgccaaaggacatatcctttctgtggaggaataaaacaattaacaaaaacagcatgattgtataacctgaacaatgaatgaaaaatgagttgaggctaaattttattctgggagttaatcacgactcacagaaaacactggaccagcttcctaaactttctgtgccttggtttgcccatctgtgaaatgcactctctgtacttcaaagttataacaatcatatgccctagattttaaaattgttccacaggcacctcattcaaacattcaacaatatttattgagggcatactattgtaatgcctaaccttgtttttactaaccctgtttttagattctctctttcctttaatcacctagccttgtttccacctgaattgactgtcccttagctaagagagccagacagacttcatcttggctctttcactggcagccccttcctcaaagacataacttgtgcaagctgactcccagaacatccaagaattcaattaactgataaaatactgtggcgagcaatatccgcagttcccaggaattcgtccaattgataacgcccaaagccccacgtctatcagtttgtaagagtcttaaagcccctgcacctagaactgtttactttctggtaatcatttatccttttaactttctgcctactttacttctggaaaattgttttaactagaccccccctcccctttctaaaccaaagtataaaagaaaatctagccccttcttcagggccaagagaactttgagcgttagccatctctcagccgctggctaaataaacagactcttaattcgtctcaaagtgtggcgttctctctaactcgctcaagtacaacactatgtgcccagcactgtttgtacaaatccaacacatcccaccagttgctcgggccacatccctgaacccaacctttgcttcttcatttctcccagatgctcaatcagtgaatcctataggctctatcttttcaatagatctagtagcagaccactactcaccactccactatcaccatgctggccccaaaactatcaactcttgcccagactactgcaatagtttccaaactgcctccttccttccatcctgatcatctacagatctcttcatacagtattcagagcaaaacttttctatgtgtcacctcactggcagacctggagtctctcagctacctttcttagctgtattttaggtaccagacttagtataccaacagtctacctggcttatagctaggactctatcatctggtattctgttacaacaaatgtactttaagttaaaaataataaacaggcttatatttaagtggcaagtgcttgatatggctgctttagcagataagtctactggtagaatctagaggagaggaaataagtcatacatggagaccaagatgcaaaaaccactcatgagcagccacataggacagaggtccctctggagaagccaccaaaggatataaatctctcttcaggtttgttttgagaaaacacccaagcaggaaagctgctgtacaaaattactattgccccattatgcgattgtgttttacttttgtcttagcattaatcctaccttgtggggaaaagaaagagagctcagactgctactgtgtctgtgtagaaagaagtagaaataagagactccattttggtctgttctaagaaaaattcttctgccttgagatgctgttaatctgtaaccctacccccaaccctgtgctccctgaaacatgggctgtgtccactcaaggttaaatggattcagggctgtgcaggatgtgctttgttaaacaaatgcttgaaggcagcatgcttgttaagagtccactccctaatctcaagtacccagagacacaatacactgcggaaggccgcagggacctctgcctaggaaagccagttattgtccaaggtttctccccatgtgatagcctgaaatatggccttgtgggaagggaaagacctgaccgtcccccagcctgacacccataaagggtctgtgctgaggaggattagtaaaagagaaaggaaggcctctttgcagttgagataagaggaaggcatctgtctcctgctcatccctgggcaatggaatgtctcggtgtaaaacccgattgtatattccattgactgagataggagaaaaccaccttaggcctggaggtgggacatgtgggcagcaatactgctctttaaggcattgagatgtttatgtgtatgcacatcaaaagcacaggacttttttctttaccttgtttatgatgcagagacatttgttcacatgttttcatgctgaccgtctctccactattaccctattgtcctgccacatcccactctctgagaaatgcccgataatgatcaataaatactaagggaactgaggctggtgccagcgcaggtcctctgtatgctgagcgccggttccctgggcccacttttctttctctatactttgtctctgtgtctcttttttttcttaagtctctcattccacccgacgagaaatacccacaagtgtggaggggcaggccaccccttcactacctgatttttatttattgcttgtctcctccttttaaaatgtaagatccaggagataagtggcctctatcttcagtaccatagagtgcttggcacatagtatgtaattcagtcagtgtcaggcctctgagcccaagctaagccatcatatcccctgtgacctgcacgtacacatccagatggctggttcctgccttaactgatgacattccaccacaaaagaagtttaaatggcccgtctttgccttaagtaatgacattaccttgtgaaagtccttttcctggttcatcctggctcaaaaagctcccctaccgagcaccttgtgacctctcactcctgcccgccacagaacaaaccccctttgactgtaattttcctttacctacccaaatcttataaaacgaccccacccctatctcccttcgctgactcttttcggactcagcccacctgcacccaggtgaaataaacagctttattgctcacacaaagcctgtttggtggtctcttcacacggacgcgcatgaaagtcagtatttatgaatgactcaagacacaaaaatagcttcataaaacagtgctttgcttgagtttttatgaataaaccaatctgaagtcatcccttttctagctcagaacaaatttctcccttttattttagaggaagatgagaatggagggtacaaatttaacatgagtttactgaagaaggaagcaccaagattaacctaaatgagaatactattctaatgacattagccagagaataatatcgttcctgttccagtactgccaattaccattacaagtcccaatatcttcatttacaatgtggggacaattataacacctaattattggttattgtgaaggttaaataagaaaatatacttaaagcccttaggacaccacccagaacttcatcaataaatgcagctattttgttattatcatatttatattagtggtatactacatcataaatccactcaaagctgatgctgagtcacggtgacccctaactgaacacattgcctcaatctgctccccataatgcacttgagatacccactgccacaatgacgtctttggtgattttaatttactactattcagaggttcccaattttggcctacaggtcacaggcagtaagaaagggatttcagggactaaatcaatttatcactaggtaaaccgaacaagaacagtttgatcttatcgtgaatcactggagggcacggaacaagtcttacttctagaacccccagggcccagcggagtgtctgacacatgatagtcgatgttgattaaataataaatgaatgatgaacacatgccacctccttgacgggcagttcaggcaatcagacgtcctgtgcgtgatcagacgcctagcgcttcagaagcacgactggtgagaactgggcagcccttccacgctccgcactgcaagaactgcctgtccggaagggtgactgcaccagctccgctccggatatcttggcaggacgcgccctctggcggcgcctcgctcgtaggtgggccccagcgcgcagtcgcgcgcccccgcgcgttgggaagttgggagggaggtgcgcgcttggccgcgcggggcggggcctctaccggcccgatggagcgcgcgggcgctactagccgcgggggccaagcccctggcttcttactgcggcttcatactgagggccgagccgaggcggcgcgggtgcaggagcaggacttacggcagtgggggctgacaggtgagcgggctccgggcggacttcggccaggcgggccaacctattgggactgcctcttgcgggccgggggcgcagcgggtgggccgcccggtgggcagtttacccgctcgcgccagggccttccttcgctcctgccgtgggcggagagaaactgcgcccgggcttggtggccacggcccccgcctgcgcggcgcgcggggccggcggacgccagatgaatgaggtcgcgggcccggtagccaggcctggcccctggcctgtggaggggaaacgtggtgagatcagcgccacctgcaggcctccgctgaagagttggacggcctggtgcaccaaggatgtaggtttccagttgctgttccggtgggtttgggtcccggcctggggagtttattggttgcttctgtaaaacgatcaactcatctcccagcttcagcttctccgtttactgtgcgcgcgcagttattggagaattcgccacggattaattctccggatcgagttacgtgcggtagtgagcggacaaactcaagcaaagcactgtttatgaagctatttttgtgtcttgagtcattcataaatactgactgaaccacgtactatatgccaacttagcttgtccgctcaccaccgcacgtaactcgatttattgacactagcccttacggagagtctgcaaagcgcgaaccttgcatgccccccagccctgccgctgcatggctgaccgtacttcctgcagctccgagaccccgctctcctcctgggtctgcgctgactcgccgctgaaccgccccagcctcgttttccttacttataagttgggaacgtagtgtgtgctttgactgtattgacagaatcatgcatcagtaataatacagtcgtttattcattacttattgaatgctactgggagcgtattcttaggcattggctacaaagatgagcaaaacaaatagggacccttcctacctagagttttagactagtgagagtgcatttaaaagtataaactaatttatttaagtgctcagtaccacgaaagagtaaggtttgtcattctaggaatgaaacaaaaggtgcaattctgtgttcagcttagaagactgaaagatgaagttgaatggagaggacgctgacatgaaagagaaagacctctctccttgattccctgagtctgtaagaatgtgtggctgtaaggagtatgtatccagttttaagtatgagcttgtagactggtctttttatgtttgactttatcttaacgaaagtttatgtttgtgggtttgcctatttccttgcaagtgttgggaatggttctttaagaacttgtgtgagagagggctcagaaaagtgtgccagttgatacttagctgtggataatatgccaggagaaacgtacatatgggcaagtgttttagtgaaaatgaggagacaagaggttgcaagtttgagtggatggaatggagtgagtaaattcagaattaagtaggcaaatgtggcaacttggataaattggtagtggagaaggaaaatagaaaagcagagtcaaaggaatggctactgaatattataacttgtaatttctatttctgtttaccagaataaactagtgttatgagaaactattcttcatgagttggttaaaaaaattcttactacttttttttcgtttggttacagaagtagtacgtattttcagtaaaacattcagggaaatagcctatgcataaagaaaataaatattaatctccataatctccttactgttaacatgttctctatcctgtataatttcttttactttctggtggagggggaaggtgaaaaatggagtttcatgtacatttttttgggaaatcataactttttttccttatcattcagtcttcttcaacatcattcttaatggttacagtttttcagtatatggatgtaccatagtttagacagtccctcttcttggtatttaggttcttttttttgctattgtaagtaacataaatatccttgtaaccaaatatttattataggtatggacgtttaattcctgaaaggtaccatttctagaataaagagtatgcaaaatttttgcttatttctctatactctcagcaacactggtattttctaatttgagaagttaatatgctatcgtattgtttaatttaatgtttatttggttaccaatattgatggacatttggatattcatctttggatcatgaagttaccttaggacctttttgtttctggaatatgcagacctattacttcttgctgttttgcttgctttttcactacttgtcatctccctgacagaagggcaaaagaatctacatctggaggttaaaaagctaaagactacctttcccagaccccactgtagtttggttgtaaacgtgacttggctttagccaggcacgtgactgggagatttggaaggggaaagtgaggggaaggacacagaggggtttggattttccgcttcccacttagctactacctcatgggtctgtgggagggtacagagcattcattttgttatcatggattgtggctgcgttgataggtccctggggctgacagtaccgtggcctcctggttggttcctggcttccaggtcgtggaggtagatacttccttggtgtgtccatactgtggtgcttgatttagcagttgtacccagaagatcagcctagatgttactcctccaggcctttcgacaattttgtggtgatctaattccctgtattacattcctttctgcctaacctaccaagggtaatttctggtttttgctgttgactcctaagtgttaagtattgttatctttgtggatataattacatattatttttgaaaattcaactttttttttttttgagataaggtctcactctgttgcccaggctggagtgcagtggcccattgcagcctcgacctgggcttcagtgatcctcccacctcagccttctgagtagctgggactacaggcatgagtcaccagttttaagaaataatacggaaggatcccatgtaacctttacccagtttcccctcgtggtcatatcttgcaatgtggcacattatcacattgtgtacacttgcaatgatggtacactatcacaacaggatattgacattggtacagtcaagatccagaacattttccatctccacaaggatccctcaacttgcactttgatagctacactcacctcccttctacctcaccaattccttaacccctggcaaccactaatctgttctccatttctataattttgtcactttgaaaatgataggtgagtaaaatcatacaatatgtagcctttggggactggctttttttcactcagagtaattctctggagattcatccaggtcgttgcacgtatcagtagtttctttttattgctgagtagtactccacagcacagtataccacagtttgtttcaccactcacccactgaaggatatctgagttgttcatagtttgtggctattgccaaaaaagaaaagaaagatattgtaaacatttgtatacagattttgtatgaaaataaatcttcatttctctgtaataaatgcctaggagtgctgtgagtgggtcatatggtagttgcatgtttagtttttaaagaagctgccaaactgtttccagagtagctgtactattttacattcccaccagcaatgtatgactgagtttggattctttgcatccttgccagcatttgatattgctacttttttatattgactattctaatgtatgtgaaatgctatctcattgtggcttagatatgaatttccctattggctaatgaaatatgtaacctctttgataaaatgtctttttctgtcttttgcccattttaaaataggatcctttgttgttgttgttttttcactgttgagttttgacatactctagtctttatataatctagatactaatattttctcagatatatgtcttacaaaagttttaaattttggctaaaatttatcagtttatcaattttttctcttatggatagttttcttgttgtttggtgtcaaatataagaactcattggctattcccagatcctaaagagttttttcctaaaagttttacagcttcttatttaagtccatgatctactttgagttaatttttgttgcacaaattttgatatgttgtattttcatttttatttagttcagtgtatttatttccctggagacttcctcttttgatggactgtttagaaagaagtgtgttgtctagtttccaagtgttgagagatttgcctctaatgtttctgtccatgaattctaattttattacattgtggtcagagaacatactctgtacaatttcagttcttttaaatgtgttggggttttctggccctgctttagtttggatatggattatctgtccccaccaaatatcatgttgaaatttgatccccagtgttggaggtggggcctaatgaaaggtgtttaggtcatgggggcaaatccttcctgaatagattaatgctctccctgagcagggagcagagagagtgactgacttcttacttactagcttccagaaagctggttgttaaaaagagcctggcatcccccacgcctttcttcctctctcaccatgtgatctctgtacatgccacccccacttccccttctgccattagtggaaacagtctgaagccctcacctgaagcagatgttggtgccatgcttcttgtacaatctgtagaaccatgagccaaataaacctctttttatttttaaattatccaacctcgagtattccatagcaacactaaatggactaagacaggccctgaatatgttgtatggtccatggcacttgaaaacaatgtgtattctcctgtctttgggtatcagcagagctgcattcctttctggaggctctaggggagaatatatttcccagcatccagaggctgcccacatcacttgactcctggcccctttcctccaacttcaaagccagaaacattgcatctctttgatccttctctagccagcttcctctctaaccacagctgttaaagtttctccgaatgatgcatgtgattagattgtatgtccattgcgttatccaggcccacctggataattcagggtactcttccatctcaagccccttaaccttgattatgtgttcagaatgccttttgccatataaggtcacatactcactgatgccaggatcagggcttggacatctttgtgagggccactattttgtctaccacttcttccttttacttttcacttatttaattatttttgggttgaatttcttgtagacaatttataattgggttatgtttaaaatccactctggaagtcttattttttttttctttgagacggagtttcgctcttgttgcccaggctggagtgcaatggcacgatctcagctcaccgcaacctcctgcctcccaggttcaagtgattctcccacctcagcttcctgagtagctgggattacaggcatgagccaccatacccggctaattttgtatttttaatagagacggggtttctccatgttggtcaggctggtcttgaactccctacctcaggagatcctcccgcctcagcctcccaaagtgctgggattacaggtgtgagccactgtgcccagccaagtctttgtcttttaattggtatacttacaccatttatatttcaagtaattattactatgtttgagcttaactctgccatcttatttttattgtttttagtttatctctgtttctttttcttgccttcctgtgaattatttgaacattttttagaattttatttttgtttatttacagtgttttttagtttatctctttgtgtagctttttagtggtcgttacgggtattgtatgtaaatgtacgtatgtgtgtataaaatcacagactactgatattgtcattttacttatttgagtaaagtatggaaacattacttccctttatataaacattacttccctgtatatctatcttccctttgtatttatagctttactttttgtttataattgtcttaaatatttcctttagaaccacatcagacactgttataatctttgcttcagcggtcaaacataattttaaaaactcaagaaaaggaaaacctattgtatttacacgtttttgaatgctgcattctcaccttgatgttccaaggttccatcttttatcatttcctttttttccaagggcttcctttagccattctttgagggtaggtttgttgatgataaattctctttgttttccttcatctgagaatttcctcttcattcctgaataccatttttcttgattacaggagtctggattgacagttcttttctttcgatatttgaaacatgttgtggcatttctttctggcctttaagatttctgacaagaaatctgcttgcatttgaatagtttttcctctttaagtaaggtgttgtttgttttttttctggctgcatttaagatattttctttgtcttttgttttcagcattttaataattacatatcttggtgtgtattttttttttttttttttttgagatagagtctctctctgttgccaggctggagcgcagtggcgctatctcagctcactgcaacctccgcctcctgggttcaagcaattttcgtgcctcagcctcccgagtagctgggactacaggcacccgccaccacgcccagctaatttttgtatttttagtagagatggggtttcaccatgttggccaggatggtctcaatctcttgacctcgtgatccgcctgcctcggcctcccaaagtgctgggattacaggcgtgagccaccgcgcccggcaatgttttgttatgtttgcggtttactcagtttcttgaaactgtagctctttagccagatttgggaagttttcagctattatttatttaagtactttttcagccctatcctccttcacctgtttttattggacaacattgaacaaatgttagatcttttgtggtagtcctgaaggtcccggagggtcatttgttttcagtctgctttctctctcttctgattgtaatctctctataacttctattctgtagagttcactgattctttcctcacttccttccattctgctgttgatcccatcaacagcatcagtagccttttattttggttatattatttttcagtttttaaaatttccctttggtctttatatcttttatttctttgctgaaatttctgtttcttacctgaggtttcctgtttttttcagttgttcaagtgcattcataactacttgttgaagcattttatcattactgctttaaggtctttgtcagataattctaccgtctgtgtcatctgggtgttggcacctattgattatcttttttcgttcagtttgaaatcttcccagttcttgatataatgaatgatttttataagaattggagccaggcattttttttaaatcatgtttaaacctcctgtttgactgtctttgtctgatgctgctctggcaggggaagagggtctgctgccttgttagtgccaggtggggatagaagtccaggctcccccttcagcctctgtccacatctggggattgggaaggggctcctccatcctgctgggtgagggtgggagttgtggctccctcctgagtctctactgatcctgcaggggaaagctaaggggtagggcctcgttattggttggtggggataaaaatcccagctccctacttggccttctcttataccatcctggctggggtgctggggcactcgttgtagctgtaggtagaagtctatgctttccacttagcctttgctggtgggaccacaggtttattcctgtggtgtttactagaatagagcagttattatataaaagtttcctgtcttgctaggctgccattttctagctggagcaggcttgtgaggggtgggggtggtatggtttggctgtgtccccaaccacatctcaccctgaattgtaataatctccacgtgtcaagggtggtgccaggtggagataattgaatcatggggtcagttcccccatattattctcatggtagtgaataaatctcacaagatctgatggttttataaatgggagttccctgcacaagctctcttgcctgctgccatgtaagatgtgactttgcccctcatttgccttccaccatgattgtgaggcctctccatccatgtggaattgtgagtcaattaaacctctttcctttataaattacccaatctcaggtattattagcagcatgagaagagactaatattgggaggtgttcttatttgttttggttttggtctacatcagttggtgtttccagttggctgatttcttgaactgtcagactgggatatataaagcaaaaataaattccagggaacttactaccctgccttccgcaggcccaaggtccctagccagtctgcttcttcactacacctttcagagttttatgcttgttttctgtagcatgtctagggtttttatttgtacttagcaagaggaataagggaaagtaagtatactcccatcagaaacagaaatctctgaattttctgattataaaatggggataatacctactccatagaatcattataagcattaaatgagatactgtaatttatttatttatttttattattatttttttgagacagtctcgctctgttgccaaggctgtagtgcagtggcgcgatctcggcttactacaacctccgcctcccgggttcaagcaattccccctgcctcagcctcccaagtagctaggattacaggtgcccgccactacacccagctaatttttgtattatttattagagacaggttttcaccatgttggccaggctggtcttgatcttctgacctcaggtgatctgcctgcctcagcctcccaaagtgctgggattacaggcgtgagatactgtaatttatgtaaagtgtttactactactctggtatttgtaagtgcctaagaaaaataacttattttttaaattttgtacaattatgtattttgaagatttttttaaaggtataagttaaaccagatagttatgtttttgctaatagttcttatataaagtatgtttaaggtctttcaccttcccaagatatggctattctttgaaattggatttttttcaccaagggaaagagaaaagagagtaagttccgtattaatttcacacgttttctgccatccctgtacacagttaaataccctttgtgaaacatcatttccattcttaaaaacagcgcttctgtgttgaagcattattcagtgtagtcctaagttttttcctttagcattgatggcatatttaaatgggtgcaattaaacaagcagacacatgtacaatccatgtgttgttgctctttgttaagttgcatcagtaatgcctcatttcccagaatggacactggtgtgagtctcaggcagtatagaggccagatcccaagttgactttctcatttatcaagtgaatcaggtaacaatgacaggctactttggggctttgaatataaaggtgaataagtctgctcaaaaagtagtttggaagtcagcagatgtttagatatccataactcctcagcaaaagatacgtccagtgaggtttagggttatgtgaatttaggctgtgttcctcattcaaactcttagaacattgcctctgcatgtactgaaatgtctgctcttcggatttgctgtattttttgtttctagggattcacctacgctcttaccagctggagggagtaaactggctcgcccagcgcttccattgtcagaatggctgtatcctgggagatgagatgggcctggggaagacctgccaggtgtgttactatgcgacgagtactgctcaccgccactgcgatacttccttataactcattctggagctgagagctctggagctaaaacaaagctcagtttcacaaatgtccctgggatccaggctaactggctcttgcaccgggaaagggccttccctgtacagtcttctctgcctcagtcattgcagttcccctactgactttattcagggccagcaaatgctacttgtcctttctttggatgttcacatagctctgctttaagctctctaaaaagatatcacctccaaatttgttttgctaaaattttgtttagactttttgcatctatgttcatgaaagacattggtctgtaattttcttgtagtgtcattatctaattttagtattggggtaaagctggccttgtagaatgagttgagaagtatgcccttctcttccattttctggaagagtttatgtagaattgctgttaatttcttccttaaattcttgctagaattcactagtaactccacacttgttttgtagacacatctggtttatagtaataaaagataaactttctctaaattgcatcctcagggaaagctagactgaatggttttaattcaataagccacttattaaagaatggttcctggcacagcttgggctgagaagccatagataatttaaaaagaaaattatttctgttataaaaactacctaccaccctgtaatcaagcactctaaccataaccatgagttgcaatgcgtgttttgcatgattgaacttttgtttttgagacagggtcttgctctgtcacccaggctggaatgcagtggcatgatcttggctcactgcaacctctgcctcccaggctcaaggaatcctcagtctcctgagtagctgggactacaggcgcatgccaccatgcacagcttatttttaaatttttttgtagagatgaggtctcactatgttgcccaggctggccttgaacttatgggctcaagtgatcctcctgccttggcctcccaaagtgctgggattacaggcgtgagccactgcacccagcccatggttgaaattatagtgcgtatatagtttgtattttgttaatctaacagtgtcactgtaattttttacttcgttatattcttcacagtcattatcaacattgcataatattccatcaagagaatttataatttacttaaatgttctacagacgagaaatggtgattcctcccctttttgtgctgtttaatcttgataggaacatctttgtgcttgtagctttctcaggattttgaattatatccttaggacagatttttctcagaaatagctcagcatttgaagatggagtctcttgacacatttttgttttaaaataggttattttctctgtatattacagcaacattcaagtcataagtgtgtactagaatcttctgaagtatgcccatttgcctttaccaatatttccattttatacccttccttaagcttaggatcgtgtattgtctgttttccccgttagaatgtgtcctccaggagggctgggcgttttgtcggttctgttcactgttgtataactggagcataggacagtgcctagcaaatagaagacaccctgtaaatacatatggaagaaaggaagacagtaggggaaggtgggaggaagtgagggaggaaggaaagcatcctccctcactcgggaaagcctggcaggcagcagagggccaccatgcgattggccgtttttacagtcatatcttggcacttcttgcttaatgttttcagagtatcgcagatcttggccatcagttggattttcattgatttctattgtctttcctgactttttctttacagtagaggttcaattacctaaacattgagcctcattgcttgttaactactgaagtaattgagttccataaatttccgtgcaagtatattgaggcttacatgatttcgctctacgaatggattactcccctgatatgcggaagttcgtacaatatttctttgtaaaacaagtcttaaacaagagtgtgtgttccctacagggttgtgggaacttcatggttgtttctcatggggaaatgtgatcaaaactgcctttctttttctgtgttccagactattgctctcttcatttatttggcaggaagattaaatgatgaagggccatttctgattctttgtcccttgtctgttttgagcaactggaaagaagaaatgcagaggtacagagtagatgtagctgaaattttattgtttatcttgattaagattttttttctggatgatgtataaaatatgataaaacaacctattgtcgtaattagtaagtttattccagaaaactttgagctgatagagtgtaggtagacactgaggatataataggggaagagtaatattattactatttggcaatttaaaggtcagcaatcgtttgtagtaagtattgatgaacttagtagaagccattgttttttgtttgtttgttttgagacagagttttgctcttgttgcccaggctgaagtgcaatggcacgatcttggctcaccacaacttctgcctcccaggttcaagtgattctcctgcctcagcctcccaagtagctgagattacaggcgtgcgtcaccacacctggctaattttgtatttttagtagagaccgggtttctccatgttggtcaggctggtctcaaactcccgacctcatgtgatctgcccgccttagcttcccaaagtgctgggattacaggtgtgagccaccgcgcccggcctatttttcatagtgacgtaggaagtaactcatgtggaagagatcgttttatttttagagtcagcacaagacctttttagatctgatccctctacctgttcacataggaactcgctctgaggttcaaccatttttttagataagattcagagccccaagactctggttgtaggacctcatgagttctgtacattgcaatcctcccatgaaatgtaattttccagatatgcacatcctgtcacatggatctagtatttatgtttatctacttcttttcttggattcagatttgctccaggtctttcctgtgtaacatatgcaggcgacaaggaggaaagagcctgccttcagcaagacctgaaacaggagtcacgttttcatgtgctactgactacctatgaggtattcattcgtttctctatagcgagaactcctaacctgtgaccttagaagttgtagagtctgctgaaattatatttaagttttgttgagagcacacacttttctgggcagggagtctaccttcatcagattctcaaaagagggctgtaaccaaaagaagtgaaggatcattgtgcttcagattagttcgatcttttcctttcttggtggatcaagggggaaggcttctcaaggaagtggcacttgagctgcctcttggttgatgaacagaagtcaggcaggcaggcaggggaaagggttttgtggactgaggaatcacgtctgttactggaggataggaatggaagacagctccggccttattttaaatccttgtttttcagtctaagacagtgtgtgccactgaccttccacttaatcaggcttttctctttgtttttaagatggcgctacttagaaattattctcagaacttttttttacttagtgaacaaatgagacttagataaatcctatagtttaagagagttcacagaaaactagcttatcaatatcagagtttatcaatgccagcctttataacgtgtcttcctaatttttcagatttgcttgaaagatgcatcatttctaaaatcgtgagtaggttgtactatttaagaacttgggttgaatgtattatgaatgtcatgtctttccttcacgttttagtactttgcctctcctggcatgtctggtatgtcttccatgagttctgtttatgggtaggcggcatggtgggagtcctgtgtttacagtcctctactcattagctgtgtgtccttgggttagttatttaatctccatgaacttcagcttcttcatctgtaaaatgaggataattgtttcttacctcaaatagctgttacgaaaattaaatgagattaaatatactttgtatggttaatagatattaggctctttacatgcaacttgcatagacccctttcagtactaccatttggagagtttgctgtaatacagaaggagaaccatttgagctgtttgctggacataacctaaaatagcaatcagtgccgtggaattaactttttagaaagggagttttaagtgtacctctaattagttaacctcatattggcccatgaaatcagaaactcagcaataccacctaataatgggaatgataggatcatgtcaagataacagttacaatgcagattaaataagggctagagtttaggtaagaaagatatgttgacagggtttcattctctataacctctgtagttattacatggttaggtggatattctgtattttaatattcaaaaatctttgttttcaaagtattttatcaatattttaaatgttatttcttatccaggttcctgtgagctggatttctattttcatgttattttgaaatactagaggctaggtcatagatttcatgacttctatctagtatttcatttaagtgagcatattatcttatttttcttaagatatacattccctctctttttattattaatattcaacttaatatttgttgaaagtcagtcactggaaagacattgttctgagagttattggcaatatcaggaaagtaaatcatagagcttccctaagaagacaaactccagtggagggatgagaagtgtacagatatccataatacatagcaatatatgggaagtctcaaaagataataaaattgggacataaatgttgctgggtactttacataaattatcccatttaattttcatgaaaaccccacgaggcagctattattcattttacgggtgaggaaaataagagatttggtaacccatccaaggttacattgctgatgataaatagcagagcagacatttaaacccagcatttggtgctgtggagcctctttttaagagaacttctcaaaatagctagttgtactggagttttacattattcagcagaaatagaatctttctatttcagataatcggttttcagtgcattttcaggtagatttaaaaacctaagtaacagagggacatttataatgctgtcctgtagtatgaatcccaacaacatagatacattctttcaatatatttggaaggttatattgcttattgctgtattgtacattctgagaatagcagggaagtgtaatatcatctctgccctaaagagatttattatggagagttaaggctgtgcatgttacaaatatgaaaaatttgaaatgttttggacaatagacttgtaaaactctttggatcaagaggattagaagttacctcatccaactttccattcagtgctggatttcccccatcttttcctcttcaggggacatcatttagagtatcctttgataagtgatttgacccacttcctttcatgagccaaaatccaccactctgtagcctgtttcactgaacaagcattttttggacacctaaatgtctagttcttcacaagggaataggacctaatctgttttgaaagctaattcagacagagccaggcaccatcctagagaaacttccataccttatctcatgaccactgtgcaacttcaactggacctttgtttcttgtcatccttaaatgcatcctctgctcatgccacccaaccttctccttcgacttcctgcactctctttggaccctcagtcctccctctactcgcttctctcagtaggtgaatggtaatgtcatagggacctctgttcctctgcctgtcctctggagtttctctgtagcctcaggaagagggcctcctccttgtaaggtgaacctctgctcaagatctttctctaattttggaggaattttcctttccatacctactatttttccagtgttctgttttacctgtatatacatttagttttttaaatatgaaaataatgtaatgggattccagaatgtttataatcaaaataaaaagttaaacatcttataattttcactttattatcttttgcatggctttcacatttgtaaaagaggatacatgatatttatatcttttttattattctataggccttttaaattgcaacataatcatatttattatttaaaatgccatgtaatattttactacctattattggacatttaggttattttccattttttgctgttttaaataatacaacttgaaacattcccacatatatctttttctgtattttgaatttttcttaaatagcttctcagtagtatctgtcaaagtatttgcttttatgactgaaacttcttgagaaattgctgatgtgacacagtatgctacaaaatgtgctctggcaacagccactaatgacttccatgtcaacaaattcagtggatatatcttcctggacatctctgtgagatttgactctgctcaccacttacccattttaaagtcacacttcttaagttcctacaacaccactgtctatcttgatttttttcttctgtttgaacatcagctctgtctttatgaccttcaccaagtcacctaacctttctgagctttagtgtctttattagtaaaatgagcacaattgtctgcttgctatactcttttagactaaataacacataaagccctgaggttagtgtctggcacaaagtaggagatcataaatgtttccttttcctttctgtctctggcttcttcctttctgcataggtctttcccattttgttaaaaaaaaaaatcccttggttttactaccttatccagatattgtattatgcacatgtagcctctcaggaaggtaatttggtggcatttgtaatagaaggggcttactgttaagtctttttaataacagtcacagttttgtagtaagacttttgattgtgaaatatgtgtttaaattacacaaaactgaaagcttgggttttctctcacagattcccttggagtgttcttgttgtggatgaagctcacaggttgaaaaaccaaagctccctgctgcataagaccttgtcagaggtaaacttacagtgtagccttagtttttatataaccccttctttttaaatatacattatattttagagtaattttagattcacaacaaaattgaacagaaactacagatgtttcccatgcatatgtccccacacatgtacagctgtcccctgtccccacacttgtacagcttcacccattatcaacataccccaccagagtggcacagttgttgcaactgatgaacctacattgatacatcgctatcactcaaagtccatagtttacattcgggttcactcttggtggtgtgcattctgtaggtttggacaaatgtacaataccatgatatctactgttatagtatcatacagagtagtttcactgccctaaaaatcctatgtgctccacatattcatcttttcttcgtaactccctttaaaaaatactagtttaggcctatatagagtcaattaaattgaaaccttttttcgagttcgatttctgcagggctaaatgaacattttatagaagacagaagaagtactaaatatggcctaacttcttctttcttttatattggagataggtttactaatatctggtgaataagaaccctaccccaatagaatgcattttatttcagatgtttcaactctcttttgattatcttcaaaggaacaatttctcttaaaaaatcttattataattcttctttgtgcaatagtagatatatcagacatgttgtacccttccccccaatttacctgttgaaaaaatttgatagttcacctgggttcatgaagagaccaattacatgctattgaatattacctccagtttgtcttgtctttgtcctacttttgagcataatacacttgctttcattcctttctctggatctcttgcatcattctggcaaagtagatgagaaataccattgtaccctagatgggcccttttttccgaggagtcagtgcgatgtgaaataccctttttattgacctggtaaagatttgttcattgatgagaccacatatgttaatttctgtgatgataattgaagtttggtccttgtcctataataaaccaattaataaatttagaggtcacttggaggaaagtcttagatatgaattctatttttactggtctgaaagttgtagtttttagagtcttaatgtagatacgatcactgtgtattattagcccagtctcaaaggtcgctgtcccctggtggggccccctctatccctggtgtcctttgctttctttgtagggacttttaacagtatctccttctgagagcttgtcttggtctgtttttcacagactgggtaattcatatgagcagaaatttatttatcaccgttctagaggctgggaagtccaagatcaaggtgccagcatttggcaagagccttcttaactgcatcctcacatgacagaaggtggacgggcaagagggagcagaagagcaagctatccaaatgctgcatgacacttttttttttttatatataaaggccttaatcttattcacgagggaaaagttcttatgaactaaccacctcttaaaggcgctacctcttaataatattacattgacaacacctgaattttgaaggaaacacattcaatccatagcagttgtcatatcctggcatctaaccttatgaaagatggcttcataaactactgtgccagtttactaatttaaaacgggaggagagaagcaggcatagtaaaagaacctggatttggagtgggaaagctaagttctgttgctggccccagagccttttcttgttattcataaggaaactaaggctcagggattaagtgaagaaatggttctgggtcatctaagcattcctttttagatgaagcttgggttgcagataactagttggaaagaaaatacatgtatttattgggctgagatggggagggggatactgccgttttttatttccccctaatattgttttcagtttataaaagttggacgcaaccagccgggcgcagtggctcacgcctgtaatcccagcactttgggaggctgagatgggtggatcacgaggtcaggagatcgagaccatcctggctaatacggtgaaaccccgtctctactaaaaaattcaaaaaattagctgggcatggtggtgggcgcctgtagtcccagctacttgggaggctgaggcaggagaatggcgtaaacctgagagatggagctggcagtgagccgagattgcgccactgcactccagcctgggcgacagagcgagactctgtctcaaaaaaaaaaaaaaaaatagttggaagcaacctaaatgtaaaatatagggaattggttgtacaatttatgcgacattcatgcagtgcatttgcaaaaggtaaggctaccaagaacaattatgtagaagaatatttaataacatggaaaatgtttgcaaagtattttatacacacacaaaaaagcttacaaaatactatttacaaacagagatggtctctgaatctttacccagttataaattttgatcccaaaatggacctaactgaatcaaaatgttaatttgtgtcatagggtaagttacctgtagcgactagcagccttggtttcctttgtgacctcacagccttcattcacctcagctctttacttggtgaacacatattgtaagaatgtgaactgatgattggaaacattacttttgacaagttcccatacttgaaatactacaaaaacatcacctaacaagcagaacaaccatgaatgggtagacattgattagacatttaaaaagaaacaaataaaaaagggagatggcaaaaaaaaaaattgtttacatctgttttcattgattgtgttattcatttatcattttttgtattataaaagcagtgtcttcctatggccccccctccaaatcaaaatatagaaagacaagaagaaaaggaaaacatcccagtaatcctactcctacattaacactttaatggtttaatggtgtatgtgctgccataatctttgctgtgtgtatacattcaaaaagtaatgtatatatgcatatatattatttaaaaagtcaaaatgtatattaaatatcaaaatattgtgtatatacgtgtatacatacatgtatgtaaatgtgtatatacatatgtatgtatgtgcatagatacacttacatacatacatatgtatatatacgtttacatactatgttttgacatttaaaacaggctgtaattacaggctcacacctgtaatcctagcactttgggaggccgaggcaggaagatcacttgaacccaggagttcaaaagcagcctgggcaacatagtgagaccttgtcgctataagaaaatttaagaaattagctgaatgtggtggtgagtgtgtgtagctccagctactggggaggctgaagtgggaagatcacttgaaccgggaggaggaggttacagtgagccgagatcatgcctctgtactccagcgtgggtgacagagcaagaccctgtctcaaaaaaaaaaaaaaaaagatatacatacacaagatgtcaagatatggcttcctcattttgatgtattgtttaattctactaaattcttgtgaatgtcagtttagagaatatcttttgcttgacctaatatcttttcttctttttcctgaccttctacttcatgtctctcttactcttggtgttcttctctgttgttcaaaatttaaggacattttttttccatttgagattctctgtgatctccagagacaccagaaccttcctaaccttctacttcatgtctctcttactcttggtgttcttctctgttgttcgaaatttaaggactttttttttccatttgagattctctgtgatcaccagaaacatccagaaatcttgacatcttgcatcttggtgttcttctttgttgttgaaaatttaaggaaattttttttccatttaagattctctgtggtgctgtgtccagaaacatccagaaatcttgacatcttgcatctgatgcaccattaaattttataaaaggaaagtctcctattataaatcttacttattgcttgcagtggtggggcctgatgctgtagcgttggattctcaaactgcatgagcatgtgcattgtgtctcagatacctcagtagactccccgacacaggcagtaacacatagtttgaatccccatctaaattcagtaataacagccatattaaattctcatgcaatacttcagagttcacaaagtgttactacatccttatataagtgttttcttcacaggattattgtccccttcttatagttgaaactgaagaggtattatttcatctgcatcaaacagctagtttgcagcttcaacctgagccatctgatttcatgtcccctcagtcatttcattaaatcatgcctctctctgtgtgggtaaaggttgtgatgggtaactcagccttgcattccagtgttatggaatttttattttatttatttatgtatttgagttctcagtagtcttcagtctcctgttgaccggaactcccatccagaacagcctccaagagctctactccctcctcagttttgtggagcctgatctcttttccaaggaagaggtgggagattttattcaacgctaccaggatattgagaaagaatctgagtcaggcaagttcctttcctgcaaatcatccccaagaagccttggcacagaaaccatcctcatgcataatggttataggtagaaaagaaggagaattgatgaccagaggacaccttccagggagacagaccgctgatattagggagatgttaagtcacacatgttgttcccagttgtctgctgttcatgcctctcttaattgtttgctatttgattctgcagtagggcttctttagttcatttttggaagaaatagaaagtgcctgctgatttgcagacttttttttccaacttgtaatttctataaaggctttgttaactttataagtcacttcctgagggagaaaagaatgtgggtgctgtagtcccaaactactgttcagcatactacagcactggtatttcttttaatgctgcaccaaaaccagaattctgggatgggaacccttcctcattcatacagccaagagttgtagtcttctgttcttgtacctttgcccctctgtgttgtaggattatccatctatccctgtgatattatcctgggatgatttttcaaaacaggtaggaggtatgccaactagtgagtttgtatgtgttgggtaagtatgagtttgagggggcttctcatagcaaaaatctccagaccatagactgaagatcacctggcgaacctgctctgattactcccatgttttgggttacctgacaaaatataagacttctagtcaaatgcatgacatacttgtattacatgggacacacttgtgttaaaaagttattcattatttatttgaaattcaagtttaactgggcatctgtatttccatttgcatatctggcaatcctacaggtagtataattctaatttagaataatttttgaaattcaagacatctggggaaagaagggattttaagtcaaagagccaaatttgaatgctggccacattcacatccagctgtgtgactttggataagttgcctaatttctgagcctcacttaacttagctataaaaatggggacagtattcctcacttgaaatttctaagctgttatgctgatcaatgagattaaacgcaaaaatattctggaaacaaaacagctttgtgcaaatgagataagaagttatttgagtgttcctcgttcttgggctaagaacaagtcatgattccagaaaaaagatgatcccaatgaaggaagaaatactataaaaaaatgatcatactggcctagaatgcaaaataagcgtgaaataagaaacaaaaataaatttctttaagttctctagggttcattgccttggttctacttttgtcccacacttcttgtatttttttttcttatgtagcaagtgaactgcacaaactcttgcagccatttctgctgaggcgagtgaaagctgaggtagctacagagcttcccaagaagacagaagtagtgatataccatggcatgtcagcattgcagaagaaatactacaaggccattttgatgaaagacctaggtaatcagagggcacttgtccatttagaaactaaatgaggatgtgatttcaggtagtaaaatattttataatcacactcatttgtatgatcccaagaatatgggatggaattttgtattctgaataattctggtcggctacagtgggactgtggcagagcatcttaaagataacagccttggttgttgcagttgtgaaatttccttttctcccctcactcagtttttcttagtgcctgtaattaagcaaacacttccaggtgtcccagtcatgtctttcatcctcccaccctgtcagatacggtagtccaccctcattcacagttttgctttccagggtttcagttctgcactgaactgcagtctgaaaatattaaatgaagattccaaaaataattcataaattttaaatcaaactctgttgttagtagcatgatgaaatctcactctgttccacccaggacatgaatcctccttttgttctgcgtatccacgccgtcagcgttagtagcctgctctgtcatcagtccaatagtcatggtatcacagtgcttttgttcaactgatctttattttacttaaaaatggccccaaagcacaagagtagtgatgcctgcattttggatattctaaagaagccataaagtgcttcctttaagcaaaaaaggttaaagttctcaataaaaaaatgaaaaacaattatatgctgagattggtaagaacaaatcttctgtctgtgacattgtgaatagaatattgttataattgttgtattttattatgagacgttaatattttactgtgccaaattaaactttatcataggtatgtatgtatgggaaaaaacacagaatacatatagggtttggtactatccatggtttccaatatccactgggggttttggaacatattccccatgggtaagggggaactgctgtatttaagagagtgcaaaacttttttgttgaatcaaattcactgggaggaattggaagtgacaagggaaagatagtgaaataatttctcaaattgcacttttttgtcccttgactccacaacaacagttaaagaaaatttagaatttgcaaaagagtaacagagtacttctgagttctatttacagttgagggtctttcttaaaacaaaatggttgagaaaattttatgtgaacatgctgttaattctcaatacaattcagtgaaatttgggaggttagtataggttcaaaggatataattgaaatgattaaggttacttgtaaaaactcagggttttggtttctgttttgttcagtaggccatctctttctgtctctctctttttttttaaatttcagatgcatttgaaaatgagacggcaaagaaagttaaactacagaacattttgtcccagcttcgaaagtgtgtggatcacccatatttgtttgatggtgagacagtgccttttccccccacattattctttggtaatgtttctgtggccaaatcataccaaaattcttcaaaataattgcatatacttactttgtctactttgtttattctcaatttctctgtattggtattaactcatatattcatgttcagatatcttcagttgtcccggtaatatcccttctggctatatttttctttttttgttaaatccacgatccagtcctagatcctgcagaccctgcattgcatttgccatgtctctttattcttctataatctagaaacattcttcagcgttttttttctttcattacatgaagagtcaagaccagtggttttgtggaatgcatgataagctgggttcttaaaaatcatttcttcttgattagatttcccattgtcttgaattgactcagtcagcctttcctcaccgctactccaggttcactaatgatctccctgttgcccaaccaatggttatttgttagttcacatttcagttaccctctcagaagcctttggcacagctaatcacttctttcttgaagcactttcgtccctcagcttctgggatatactttctcttctccatctgctccttctcagtctcctttgttgcttccccttcatcatacagacctcagtaaattttcccctgggcaccgctttagctgcatcctaggaattttgatgtgtggtgtttttgtttttcttcatactggggcttttttgattccctgattggtaacccttggagcaagcactcctgtggccatggagactctagataggatcagtacagagggcttgctgcagtcattttaagggaatctctgccaaatagtgctaagaactgtttaaagattgcacaaaatctcaagtaggtgcatatgagaactttttttaagaggagggggtgttgggaacacataggttttgaaagaagtcctccaggttattctgactgccattttgacttattttatagagtgagtctcgatttcagttttgggtctccttgacctttagcatcttcttctgtctcagtttcctgaagagtggttttattccttacacagatgtttattaggcttgttggatgtgctaggctgtgtaattggtgttaagcaggactgagatcatcatgcaaacaactacttatatgatgagcttttggcttctcttcctgtagcctagctactggcttctgcccttactgagggcacattactgggagtgggttctttcttttctaggtgtggagccggagccttttgaagttggagaccacctgactgaggctagtgggaagcttcacctgctggataagctactagcattcctgtattctgggtaggtggtaggttcacatttgctgctctgagctaatgactgttaaaacctgactattgaggaactcactgagttgttcaggccaattccagttttcttttttttcttaacactgattcaggttctgccttctctgtgactacactcccaccccattctatcccactccaccccttccacaatcattctttcgtttcctgaatttgtacagcacttataatcctaatccagcacttggcaatgtgctgccgtaatctgctgtctgattaactggtgtttatgtttaccgttatcattccaactatatattgtttggctctacaaggacagagacaacactgagcatttcttttatagttgcctgctagtaacttggcattgaattgacacataatgaaggctcagtaaacattcatttttgttaacctgtggggtttgatttaaacttaaggggaacttgaaggactctttctcagggacatgagttgcgcattagaagacgaggttcagagccaggcactgtggctcgcgcctgtaatcccaatactttgggaggctgaggtgggcggatcatgaggtcaagagatcgagaccatcttggccaacatggtgaaaccctgtctctactaaaaatgcaaaaattagccgggtgtggtggcaggcgcctgtagtcccagctacttgggaggctgaggcaggagaatcactggaaccctagaggcagaggttgcagtgagccaagatcatgccactgcactccagcctggtgacagagcgaggctccatctcaaaaaaaaaaaaaaaaaaaagaccaggttcagttagtgttcaacagccatgtgttcagcttatacctaatcctcctagtcaccagagttctctctttctagaggagtctaggaaaagcccagattcccatgggtttcaaaattatccctttggaatgactgtcttaggtatggcctgaactaatctaaaacttcagatttggcaaaattgctcaactttaggaatgtgcaagttaaataatttcatgtcttactgtatttcattggttctcgtatatctgccataagtatgttagagttggagaaggacctataaatgccttctggccagttttttatttcacagacccagaaaggttatatgacttgcccaaggtcacacagccaacaaatggcagaaatgagattagaattgaggttttcaggttcattgctttctctacccatttggggcttgaatcttgaaagagttccccataatttttcctcttacacttgttgcaagctcagattaaataagtttttataatgagaatattgttttgacagtgctgtgcttctttgtttatgcaaatttaaaataacagccagtaacaagggactctaggcttgactttgttcttgacttactccatcattttgccgcctttcttccctcctctcgctatacaaaaattttctcgtgttatggaaaatgagacatcacttaccccttgcttctctaaagtaatgcttctcagacttttcaacccatatagctgtagatgagaggatagtgactttacacccccaaacagggcatagttgtagatgactgaccacaggctttcttcagagtctccagtttttcttttctttttttttgtgtgtgtatttgaattttgcattttactcttcacatatctgtatttattttgctactaaaatgaaagcttatatttctttccattgagcaaattgacattccagaaagaggcaccttgtttattctagggcttatatcccctgttgcattgacacgtctcctgggaataatctccactctagtttgaggatgactgctctgagggatacagctacctgtggaggtgtattctcatagaaagcatttggaggttctgaggcagtctataaatcatacgacacttatatttctactttggtatttatttataaacttttattgtttggtaaattttgcctgagggaaattgaccttaaataccactagacttggcagtgtttccttttctttttcttgccaggggccatcgggttttacttttctcccaaatgacccagatgttggatattctccaagactatatggattacagaggtgacaccttttggccactacattacctaaggctctgttagacttaacagtccagataggtccatgaagaataatatgggatatgagaatattacaaaggaaagcagggtgagaacattattcagaaccaaaaaatcaaaaggcgagaggagagtgatgtgtgaaggcaaggatggacagcagagaacaggcacgtgggcagaaataaacacccacgttcccatcagttacatgatttaaaattatgggccgtggagcaaatgttgtggaaatgtttttgaaaatgtgtgataaagtttcagtgactagagcttttagcgtcttgtaacattcacctcaacagttgagcacttactcatgatcagtgaaaaggtgaatattgaaattatagagataacaaataagccaggggaaaagtaagagcaactttttctgcatagacaataaagaatgtaggttattacctgggaagtctgtttaatatgtaataagatttgtgtgagatgatgagaaaaggctctaacatgagttgatcttgagcccaatgttgaacagctccagaccttacaatttaaaaaagtagttcagaccgggtgtctgagttccgcagtatacctggtccagtggacacttgcagaatgccgttggcacatgccactggccattgaggggtccccagatgcataaacagcctgatcctgtagctccccttccccacacggatgcatggaggcaggtggcgaactctaaagcctcactgaaaggcagattgctggactgttagaaggggctcactcacctgcctccaagcgcttgtcttctgtttacataagaattacatctcagcaaagttgaaactatcacacaggatagatgctcagggttgcttgagaatagtcaaaactgagtattaacttcataagtgccaaagacttcaactgcatgtatttaaaaaatccagaggagtatgttatggtgagttattttgtaaaatgataattgtccctgttaatttaaatttttccctttgggatttgcttaaagtagggctgtgcctgtatatggaaagggacaaaattggcctttggttttgggcttaattttttattccccaaagactacttgaaaagggttaagatttctgtttttcttcctctctgtaaaggctacagctatgagcgtgtggatggttctgtgagaggagaagagagacacttggccattaagaactttggacagcagcccattttcgtttttctcctgagtactagggcaggtaggctgcaaaggcattgatggaaacagacaaatgagggataatagagtactattacatcccaacggttagtacacttttttccttaattctctgaaaggtgaggttactattgaatgtaaaacaaggtactggacatcaagcatggtgctgttttctatccagcctgtccaaactgtcatctcagcaaagaagtaaggctgaaacctggggttattggaaagtaattctaatctgctttgaccattgacctgggaatgtcctgaaagatttatgtgattttgtggaatgtttcatttacattcagtggaagtagctcttcttcccaaccgtgaatttgggaaataaggtaacagtttgtctactagttgtccttcctctataagtatttctggaatagtgctgaaaagcttaacaaaaatctagttgttaaaaaatgtgattatgttgaaaataccaactttttagaattatttatgacatcatccatatatgatttaaatcgtgaatattacgacatttgtaatgctttaccagttacagagtgctttcatttactgttacataatttgaaatcagctcttggagatgaaatgattctctaagtcattgtggtgtctggaaaaaaaaaaaaaaaggccggcacggtggcccatgcctgtaatcccagcactttgggaggctgaggtgggtggatcactggaggtgaggagtttgagaccagcctggccaacatggtgaaaccccgtctctacttaaaaaaatacaaaacttagctggatgtagtggtgcgtgcctgtaatcccaactactacggaggctgaggcaggagaaccgctggaatccaggaggcggaggttgcagtgagccaagattgcaccactacattccagcctaagaaatttttctcaggtcctggagcaagctgaccttagttttcaactcataggatcctagtttcattatcttatttttgtagacataaatcttgatggagtacatgcaggaacatgaaagagatgtgtgtcctctattaaagacagattgacatttttctaaaaagagagttcagtcttatttagaaagctttctaaatgcctgctgctataagggtatatgaaagaagtgttagatataatttttgattataaggagattatttcacctgtgtttgttttatctccctaataaaattaataacataagattcatttggcctcactcttccaagatcatagactgcacatggagtctcagccattttctcatgtgatcagttgcctcagggttagtctcaggagaaactgaaagaatcaggcagtgcatcatcactgccgggaaaacagttttatttatgctttaatgatttcatcatcctcatattcagagagcagcattatgtttgaaatgtctaaaattaggaaaaaagagatctctgcttttcagttaatctccttggaggactcagagtagatctgggagctgaagcagtcctggacattagtcttctccaaacactgttgtgtttgctgtcacagttttgttgtagttttgcagtattttcatttatttaacaggtttccttccaaatttcaaatatttctgtgatgagtcatgttgccaccagatggcagtgatagctcatgaatatgttcctattcatggatgtgggtgtggcttatttataaaaatctcacccctcggtgaagagctgcacttagacaacatgaattcaagaagataattttatggaacacattttaaaatgaaataagcacctgaaaagtattatagtatagtggataaaagcacgggctctggaccaagactgcaagggaatgaatcctggctctttcaccttctaggcttgcaacttcagagaagtcccttaccctccctttcaacatctataaagtggggaaaatcgtagcaactactcaacttcccgacagggttgttgtgagggttaaaggagttaatatagagagagtgcttagaataatgcctggcaagtagtaagcacagcgtaagtgtcattatcattattattaggtataatttagcatctctcagtaatcggtcatgattacctccttgttccaacttcaacttgatacgaagactttaattagaatattcctgcctgatttgtctggagatccagcttatggtcagtagtccttcttaaaagttagtccttaattcaggtttatggaacaagccctttcaggcttgcttgtttcagcaaccagctctaacgaccctggcaagagggagtctgttttgtacttgttttcacattaatcaaagagaaggctgcaatgtaccttcacggttctcttaattaattcctgtaactcaaggtacctcctcagctctcttcctgcagcactgaagaaagaccagcaagagtgttctgagcaagcctcagaacactcagagtaaatgacaagagtgttcttgtcttgccgttggttttgttactttctttttgattaatgtggaaaccagtacaaaaaagactcactggagttttctctaatcagagggaggaggtttcccactctgctcaggagtataatatcatccactcttctcattaactttttatcagagatcttgctacctagttgtaacttgcaagcgacattcggcactcttctcttgacagtgcgcactgcagacctctcatatttagatctgttttctgaaagagcatgtgtccttttcctcagactactctaatcaaaatctaatcaaggtttttaagcagaagagataaagtggctccatggcactgacttaagtatccaccttggccacttgcccctgctccgctcattctgttccattcagtaataaaaattttcccatcaggcaataagaggtcaggtagcacttctcaccgctggaacaaggctttggagttaggggtgtgggtccatttgaaggatgaagccaattgttttgactgatttcagtttatcagtctgacccactctagccttgtgcttattttctagctcctcgtctttgtgctgctgattacattcctttttgcattgttttcaggtggagttggcatgaacttaacagcagcagatactgtgatttttgttgacagtgactttaatcctcagaatgacttgcaagcagctgccagggctcatcgcattggccaaaacaagtaagtgatttttttctgcttccttggcttgcccagcagcagttctgggttgtgaaaaaggtgaagaatatagtcctggtgacagtcccacactgggagctgagagaccaccaggttttagctcatctgtgctattgactcctagggtagtattgggtgggtcacattatcagtccagactgactttattagaaggagtcaaatcaaactgtgaaaggattagaaggaaactttagaagtcatttaactcatccttcttgagttagggtctgactcagttaaaaaatggggttatggggctatggagctaagctaaaaaaaaaaaaaagaaagatagatgttgccctttgatctgaggataatttgatcttccagatattttccttggctacagataaggaatcccagtcatggttaccccatcattctttctttgactgtctggaatggttcagagagaatttcaggcgagttctctctaacaagtgctcaggaccaaatgaaccaatctccctttcattgtaccctgaatatggtatttggttttgtttgcttttagatgtatttaccttgcatacttttgcccagctttgcacacccttatagcacactacccttgtttgacttatgtccaggtctgttaaagttattcggctgattggtcgagacactgtggaagaaatagtctataggaaagcagcctccaaactgcagctcaccaacatgatcatagaaggaggccattttactctgggagcccagaaacccgctgccgatgctgacctccaggtatgatatgatatactgttcttcactttggaatataccaataccctttgtggaggagaatgtaaatgaaaagaaccagcactcaccctctccccagctacacatttgttccttggcctccctcacacctgccacagtgctggctgtgtgcagggtctgtaggaagtaaggattagttccaagcctcatcacttcttggctgtttgggtttgagcggctttcttaacttcttagatctactctttttgcatttctaaaaataaagacaccacaggttagctcagagggctgttaagagaattagttaaaataaagaactcaataacaattaattctgtacttccaccttagtcccagagcctttgatcagtgacttacattacttcatactcagaagagggcgaatgagatcaggaattcataattgtgccttagaaaaaatgggtgaaagaactagaggtaatttatttaaagaagggagtactggatgggagacagacactggattggaagattttagagctctcttttggaagaggacttagagttactctgtagcagcccttgggttaaaattaaaactcataatatttcctggatgctttgtttttgccctaaggatgaggggctggatgcaaagagaccaactcctaggatactagaaagatgcaggtatgaagggagtaataaatgtctgtcaagggcagcatcagtgggagagtctggtgtgagaaacattgcaaaagaaggaaggacaggagttggctactgtttagagttgggtctcaacagtagggagatagaaaattcaaagatggctgtgaggttttaggcccctatgatgaggagagaagaaaggaaaataagaagtagggcagagttttaggaagataaagagaatttaggctttagtcagagtgtgcagtaaaaatacaatataaacaaactattgttagaggcagactcagacaaaaggaaagaattttatttgtaaaagtttgcaagatggactaggattggaaaggactagtccatcaaaaaacataagtgtttaagagagaaaaagtgacacaatattagaagcagagttactaagtttgtaattagtctgaaaaaacagcagttttcttacatggttaccgtatctgcaaaggccagtgcatatctttacatatcagtgttgcaaaagacagggatcctgttgtttttgttagggagttagtaattacaggaaaggctcaaggttttattaattttgggactagaactagaaagagtaacactgggtttgttctttgtttatcttagggggtaggtgtggcttttttctttttctgactttccttgtgttgctgactgtgtcacatgcatgcttaattaaccataatggtgctagggcaggctgtacattttgttttcacactaagagacaattataaatgtgagatgaaagcttgagagagaggtagaggtacgctgtagatacccttaaatgcagttttccacagaaaaattatccatagaaccttaagagagagaaggtcactgctgggcatagtgaaggggtaaatgacagagcctcacaaggcccgcattctcttgttagaggaggaaggatgtcataggttgtttgcactctcccagtggagggagcgccaggggtccaatgaggggtatcttgtgatgtgggctgctggacacatcactgtgaaagatgtagacatacctccaccccatggggccacaaacgagtgggaacatggactgctggctgagagcgactctgttggacttcttgcccagctcatggttatcggaaagttactttctgactctaatgtctgatttatctcttccccatgcagatgctatgagttatttgtggttaccaaaagcaaaggtgataacccagagcccttgtctaaaaagaaagcaggggatttttgtttgtttttgttttttgggtttttttttttttttttttttgagacagagtctcgttctgttgccaggctggagtgcagtggcgcgatctcagctcactgcaacctctgcctcccgggttcaagcaattctcctgcctcagcctcctgagtagctgggactacaggcgcgcaccaccacgcctagctaatttttgcatttttagtagagacggggtttcaccatgttggccagactggtcttgatctcctgaccttgtgatccgtccacctcggcctcctaaagtgctgggattacaggcatgagccactgcgcctgggggtatttttttttttttaaataccaagaaaccaaaagtaaaagatgtggttctgatttggtaaatctaagcagtaggtatggagttctgaagtcctgaaagaaggaaacaggttttttatcctgcagggaggacacagtagaaacaggcaggcagatgcaggtgtagtgaacacttattggatactgtgtgctgagtgttgtctgaggtgctcttttccagttgtttcagtaaataagaataacagcaggatgagatagacactatctttatccccatcttaagtaatttgcccaaggttattcagatttaggattccaatccaagcactctctaacctccgagcacatgcccttaattactgtaatatacagcttctcataaaaacacatgtaattttcttaatgactaagacacattgcaagtgagcaataacaagggagagccaggaggtgagcataagtacaagggggtgaaagggagggtcccagtatggaccaattcttatcataaatagttggcttcctactatttttggtaccagctgccaaagccagtcatcctggttatgtgtatggagggtaaatataatatatctaggtacattcatgcttaagtgagctgtctattgtttcttcaagctgttacagaataccttaacatttccaagttactcacaaaatagacgatctggagataacccagtctaaaagggcaagatgagaacaagggcccaaggtttgaatccaccttgggtcaggatctcagaattagtgcttacggaggtgcaaagttggaagtagcaagtgaaagccaggaaaaattatctgtgctttctgcatggttcctacagccatagggaataggctgagagtactccagagagggacgagagaagagaagcaggatagtgcaatgccagaggaacatccagaaaaattcaaactgagaaaaggccttcgggtctggtggtcagaagttgttactgatctttgccaaggtggtttcgatagaccactgtgttaggaaaacaaattgccaaagaaaaggagtcagttcatgatagaggtaaagttcctagtgtagccttccctttctaaggagtctggcagtggagaggttggaaagtagctaacagggtctctgatctcaagtggctgctgggaatgcttatgaaaaagtcagtgagaggtgctgtagaaaatgcaggaagttactattattcttcaaaaaaattggaggcttatacattttttttgttttgtttttatgcagaattgtcaaagtcaatacctctgataatcatttatcacctctctgcttacccatcatccaactattaaatggccctggctgttactatctatgatggggagagcagaaaggctgcctgttcattagagaaggactgtgcctggtgtcgttaatccacttagccaatcactgatatcctaatgtttcttttcatgagaatttgctggacttttttgtttcctctattcaagttgagtgagatactcaaatttggtttggataaactgctggcctctgaggggagcaccatggatgaaatagacctggagtccatcctgggagaaacaaaagatggccagtgggtctctgatgccttgcctgcagcagaaggagggagcagagatcaagaggaaggaagtaagttggaggttagagcagagcaaatggcacaaccaccccaagctagagctcacgtccccatggaaagttttggatgctgctctctggggcatcttttttctcccttaccctattgtcatttgggcacactgtttaagacttgcttgataaaagaacgttacccaaactaactggaaatttgtgtggctcttcccttgtagctgaactgtgaaccaaaatcatagtattaatgtttatgatagtatcaatcttaaggctttgaatttgtaccttttctcccttggttgcaaacatcttcttctttattagtaaagcctaccatccttggtatgatgctttgcacatagcgattcctcttctaaacagtagaattacttgtttttaaaattgcagctaacattaagcatttattttgcgttcatcaacagtgcggactttgtcatgtgctttttccatttaatttctgtaatccatgagatgtaggagatggttttgtctttctcttaattttctttcctgaatttggtcagcatttgtcattttgttcttttctattctgagcacttaaatttccgatttgaagtaatttttcacatggtagctttgtaaaggtattccctggcatcttgtagttattttgaaatgacttatttttctgtaccagctgcagcagagattcaatatggactggggtgagaggtttgggagtcttactaggcttcttaattcaccagtactttcttttaattatacacaatagtgctgtttcttcactagatggtagctcctttttattttgggtagtggtagtggcatgatttctggttttgtagttctcttttgtttctataggaccgtgaatttccatcgctcgctttctctctgtgccacaaacttgtcaaaggatgtcttcccacttctaagttgtctctctccctgccagaagcaatgccttccctaattcctggctgcatgtattttcataccttcccttctgttcagttccttagtagccactgctctgatccactcagacctatcctcattattttcccacttggaatgggactgtcttttgtgggtaacttttatctgtctgacctttctggaaccctcctgccctctccactgcatagtctctgcctgactgtctactctagtgtgggctttggagctggttttgggggttcatttctcttaacttccataagttgaagtgtgtaatattttctgactcctaatgtagtaggcatggattggggtggttttgttgtccttgttgatctgtatagtttttgtgggataggtggaaaagttggaatttgggcagctggcattgttttacaggaaactgctttttgattttatgttttatcttcgaaattctttataaaaatatcttgtttgtattcttcaagaactctttcttgttctctgcttattgttttaattgtaactctgttctcatttcaaggacatactgtcttctctggggacatttattatggcttcttaatatgtattccagggagaatattacatctttttaaaaagtatttctcttcccattgcattgacttttacttctacttctttaaaaaaatatatatatatttatttatttattgaaattggcagataaaattgtatttatcatgtacaacatgatttcttgaagcacatgtacattgtggaatcattaaatctagctaatgaacatacatcacttcatatggttatatatttgtggtgagaacacttaacgtccactctcctagtatttctcaggaatacaatatgtcatcattagctatagtcaccatggtacctctttttctaaaaaggaaaattcgtttggggatctcttgttctcatcgatagtttccccaaccgtctggtattccctggctgtctgatcacatgtgctgatgaagtgccacaaagctgagggcagctctggcatgggccctggggacttattcctggttggtgagtcagcttttacatggagggcaccttctctgatccatatttgatgtcttttcactgggcaacccattttctccagagaccaatcttctagtattttccctgggagaggtgagaatggagttcacctggttgctgaaactgaaaaggcggggtgagtcaagggctcatggcactcctgctctttggggtgcagatcttctctcaattccccgctttgcagtactctgtacttgtaagtcctaagctcttgggggattgagagggtctctagactcctaatgagcccttggctaggcacctgtgttttgtttccatgtctcttcttaatctgtcattatccctccagcaactttgcattttccaaaaggttcttgaactttttcatccaccattgcctcatagatcttttttaaaattcctttaactgtcactttgtggtttcaagtgagagaagaaatagatgcatgtgatcatatttttaagttataattgattatattaagtagcaacacactcagttctgtactgatctagataatttcagcttattttcctaacgtttactagaacaaaataaagtcacactcttttccagaaagataattatatttctcagtcaatccaactgcctaaaataattttactttatttagacagtccaactgccagaaaaaatccccagttgtattacactttggaattttctcttcgatgaatggatataggtccgctctgtggtaaatgattctcctggtaggatagagacgcgggtctaggcttgtgatggcagagtgaagataggaagtatgattacaaagaatataagtggataggaaagactagtaactaacgtggccccaatcagaattaaataaaaaacagggttgctttatcttaaatgccaacatttttttaaaaagcatggttggaagttgagaattgcatgcagtatgaagctacatatgttgatcatatttgacacttctcagctctatttttttctacttgttgatagagtgcctcattgaaagccccctgctgatttaattagcaaatgccaattagaattacagctggttagatttgggtacaagtgtgaagcaattgatctcttgagaatgaaaatgttttgctttcatactctctagggaaaacatacttataatggatttcacaaatattgtgaaaatatattatttggtaacatgtgctactaaatatgcttcccgattcaatcattatcttacctatctgtggttgctagtcttggctggtcctgacttttcttaatcacttgattcatgatcttggcagatcactcaacctcattgagcctttttgttctcatctgtaaaatggtcctattaatgcctactttactcttttacacagttggaaaaatcagacacgattatagttgtgaaagtgatctgacagcatgaagtgctattcaagatgacactattgtcttcattgttattattaccacagttattatttgctagcctgttaatctctccacccttctagagacccaattatatactgaaaagagcacactggccttagaatcagaaaatcctgcctcttccagtgagaattacagagtcccttaatttctgcctaagcctcagttttccctttcaaaagtaggattagttataccaggattgtggtgaggatcatgacgaagacgcttgatgagatctgtaaagaatattgtaaatccaagggattatttttgtgattcttcattttctcatagatttgccaagctgaatattaaaagtgtgtttggaataaaaaagtacggattttattagatgatcttaatgtcagtgagatttgcgctgagggatagttgggaataaatgaatgaggaatgaatggaagaatccagcagagattcacaaaccatctagggatgaaccaaagggttttaagccatgctctccccttggaaaagtaaacacatgggatccccatgtagaacccacattcttcagtgtcagtgggatgggaaatgaaataccttccttcatatggacttagcccatttagaatataggctgttctcctgtccacttttgttattgatttgaatagcattaatctatttttccttggtatctaacatttctctctttgtgttttatgttgttagaaaatcatatgtacttatttgaaggtaaagattattctaaagagcccagtaaggaagacagaaaatcatttgaacaactggtaaaccttcagaaaacccttttggagaaagctagtcaagagggccgatcactccgaaataaaggcagtgtaagaactgttaatttatttaaaagttgttcttccaaactctcattctaaaacaaacaaaaaaatgatgctggcatcgttttgttctcttaggatgatttgtcaagaaataagtatgtgtttgctgaaatgttattataattaactataccctagtataaaaactatgtaaaaaagtcagcatgaaaaacataaaggagagaatatattgtacgatgtcatgtaggtgaaagcagccttgtccatccaagtcacccctaaaggcattcctatattataccaaaataccatatcctgctgttggtaatgatgaccctatgacaagaagagaggatggcaatcataaatgatatatgtagtgttcacagtgtttggcagttaacgtggtcattaaatgctagctatcactaagataatcatgatgttgaaatacaatcttaaaaaagttacataatacattgcagaaagagttccattaaaaatggctgaagtggcatcctgcagggtatgcttttagtcaaggaaaaaagttacttttctgaagtaacttattcctaatgaaatgaatcaaaatgactgtttcaaccatgccaatgctagggctgagtttacagcatggtatcctggtcactgtgcctgtgaagtgtgtagtatgaacagtgcctccaagtgctttgcctccagttcccaccatgcagggtgtgtggagatgcagtgttctgtggaatattaagcatgttgcttccgtacagtgtgtgttagggataatgaaattcggggaggaatcttcttgaccctggtgatggatcttgttcttcctctaggttctcatcccaggccttgtggagggatctaccaaaaggaagcgggttctgagtccagaagagctggaggacagacagaagaaaagacaagaagcagctgccaagagaaggagactcatagaggagaagaagaggcaaaaggaagaggctgaacataagaaaaagtatgtctgcgttaaccaagctggcggccacagttgaaggagtcactattgtatagtgagaccacagttgaatatcactttaaaaatacagaaaattcattttaagttggttcctattggtaacagaatactttctgaaaacatttcctctaggtaagtgaaaagtctcagtgtataaggcagggaagatgcattccattaaaaccagaattgttttcttttttcttttgagatgggttcttgctctgttacccaggctggagtacagtggtatgggcacagctcattcagcctcaacttcccatgctcagtgatctacccactataacctccctagtagctgggaacacaggtgtgtgccaccatgcctggctaattttttttattatttgtagagacagagtttcacggtgttgcctaggctggtctcaagatcctaggcccaagctgtctttctgccttgacctccaaagtgctgggattacaggcgtgagctaccatgcccggccaaaaccagaagattttaagattttattgtagctatctgacaaagaataatttacttcaacaatctcttttagtcttaaaaacaggaacattcagggagtgctcattattgaattgtagtcaggaagcagttagcctaatcagtaagacttgtttacaaataagtagaaaacttcaatcagggtgagtttctaattgcatttctacttggcagatattgtttgtgaacagcagtataaaatgtgctccaagggaaattgtgattgtctgggttaatttccttttgtctctggcctgctaaaggatggcctggtgggaatccaacaattaccagtccttctgcctgccctctgaggagagcgagccagaggaccttgagaatggggaagagagctctgctgagctggattaccaagacccagatgctacttccctcaagtacgttagtggtgatgtcacccaccctcaggctggggccgaggatgctctcattgtgcactgcgtaggtacgagaagtggtatgggctggggatgggggcctcagtccttatggtgccaagaactggggaggatggggcactgggactggggtggtggtcccagtgtagtattgtacagtcaaaaaagtgtgaattttagagtcaggagatattccagaatcatttcactcttggctttctcatttacctggtttagttacccaacctttcaacttcaacttccttatccatatgatgggacaatatctgtcttatcctctgcacaaggtttttaagagggtgaaatgaagcaacattgataagacaaacaaatcctttgagaaaaagcaaaacttcaagcttgttcccttgcttgacctttgtactttttacttcatctgcctaaaaccctttcttcccaaataaccacatcaagtgttgttcaaatgtctgtttctcagagaggtcttctgtgattacctcatataaaacaggccccatcccccctgttattctctgtcccttctcccatattttcctttatcacacctgtcccacctgacacattacctatgtatttgtttatttgactgttgctttgcattaaaaaatacacttatggcagcaggggttttttcttgttcgctgctgtgactgtggtgcctagaacgatgccttacgtgtaatacatgctaccaaacgtttgtagtgtgaatgaatgactataaatgctaagatactaagcagctttgttagtaccagcttgaataagtcacttaacctttcctgtgtactgtttcataaccttgcctatgtgctgttgcataacctattgcttctactcactctgtaatgttccatctactctccgtccttccgcagtcatttgccaggaatcacagatgcaccacagagattttgctcattgagaaccctaatttttgagatgctttcctgttatcatggccccagctatatcttccagaaaacataaacatatttgggaagtccaacctgtgatattcctaggagataagatattttgtttcttccctttgaaaaatcattcttccacaagtcccttttgtgtgcctttgtttttctaaattgtgcactggacttcacctcctatagatgaaaattttctctttcttcaaacagatgactctggccactggggcagaggtggtttatttacagctctggaaaagcgatccgctgagccaagaaaaatatatgagctggctgggaaaatgaaaggtaagaagcaaagcagagggaaaggttaagggtggaataagagagaagaggacacctaagactgtatcgtgagggttacacagcactagataaggaattagaataaccagttggggactgaattctgtcataaattagctacttgttctgtgacttcaaggcattcctttaccttttctgtacctgtttcctcatctgtgatttgtgaataatacttgttctgcctacttcatagaactgtagtaagcataataaatgtgtgtattctgaaaaatgttgatccctgcatacatgttaaagtattggaatgggctggacacagtggcccatgcctgtaatcccagactttgggaggctgaggcaggaggattgcttgaggccaggagtttgagaccagcttgggcaacatagtgagatcctgtctctaccaaaaatttaaaaattggctggatgtggtggtgcatgcccgtagttccagctactcaggaggctgaggtgggaggatcacttgagtctaagaggttgaggttgcagtgagctgtgattacaccactgtactacagcctgagtgagagtgagaccctgtttcaataaaaaaaaaaaaaaaaaaaaagaaaaagagaactattggaataaacatgaaggaatatgtcatgaaaatatcaaagatctatgggaagccgggcgtggtggctcacagctgtgatcccagcaatttggaaggccgagacgaggcaaggaattcaaaaccagcctcaccaatatggcaaagccctgtctctacaaaaaaatacaaaattagccaggcatggtggcacatgcctgtaatcccagctactcaggaggctgaggcagaagaatcacttgaacctgggaggtggaggttgcaatgagctgagatcatgccattgcacttcagcctgggtgactgagcaagactgtctcaagaaaaagacctatgggagagaaattggacataccattaaaatgctgacaagaactcgggtttggtgctgagtggaatgaagatgtgttaagaggtcagcacaaccttgggtataacactccctggagacagaaataaagctgttgggtgccaggggaacttagaagcctgaacaatattgtcctttggcacagagaagggaaaaaggcacctccttttacatccagaaataacaaagtggcaagaataaaattattattgtggtgattttctggagattgaaggaccttgtctgatagagaagggccctccagattccttagatattgttttttcctaattctgcccagttctctatggtggaaagggatataagaacttagaatgactactttttctagtaaaacaagttactgaaagaagggtttaatgtgtgttgaaatagtcaatccagatctagatgctgattgggcagttggcaaagcaaaacccagggaaggtcagagctggaggtgcagattgaggagtccctgtttggagtctgtgtttaaaatcatgtgggagagaggatggagaaatgagaggcagagaacagacctggaaaacacctctacttaggacttgaggcaagaagatggaatttctgacagaaggaattgtcagacaattagggaaccttgtgcggtattttgaggtacaagggaggaaagtatgtcaagaaggcaaagaagttcatggtattagacactgaagtgaggatgaattgggaaaaggccatggattttgacccaaggttgctcaccttggagcactttgaggagagtgggaagctcagacttaaggcctgagggctcaggaaggaaatggagatgagagtgtgcagttttctctgaaggaggattgaagcaggttgcagcaaagtaggtgaaactgtggattccaattcccagggaaggcttcatggaggtcctgggcctggaaaggtgggttgaatttgaataggtggagagaaatggcaagaggatccccaactgctcattacaacacttactattccttgtctgtgggtattgaaggacccaggcagttagcctgttcctttgtgtggaggatggcgtacaggccatgcaggccagagtggagggtttaggcagaagaatagaggagagtttcgttttcatcagcggcttgggccacatcatagaagacgtcacatgatttgtccagggagatgccattctgcgcagaaccttatctaatggaatgggtaatagctggtcgttttgggggatttgatcaaaaggatggcatagcacaaccagtattttagaatgactgaacaaaaagttcaaactggtatcaacctaaccaatagacagggtctgtaaaataaaaggaacaaaggttttttgttgttttgtttttgtttttgagatggagtctcattgtctggagtgcagtggcccgatcttggctcactgcaatatccacctcccaggctcaggaaatcctcctgcctcagcctcccaagtagctttgtaccacaggcgcacaccaccatgcccggccactcttttgaatttttggtagagacagggttttgccatgttgcccaggctggcctcaaactcctgagctcaagtggtccacctccctcagcttctccaagtgcaaggattacacacataagccactgcacccagcctgaggtttttaaggagaaatgaggaagattacatactttttttgaatcagttatccttggctacaaggattagtaagggtggcaccacgccgaggttgggcaggcagttgatgagcagatgtctttgcagaagtatatttttatgtaagcttgccagggcccttgtgcaaggtcatgggttttgtaaaatctgttgtgatagttcttgttatcagacgtttatgcattagaaccttcccttcatggccttccctggctctatttgtcagagttttgttttattttttgagatagggtctcaccctgtcacccaggctggagtgcactggcgtgatcatagctcaccacagcctcgaactcctttgctcaagagatcctcccacctcagcctcccaagtagctaagactacaggttcacaacaccaaacctaactttttcttattttttgtagagactgggtcttgcgccttgttgcccaggttagtctggaactctggcttccagcaatcctcccacctcagcctcccaaagcactgggattatagtcatgagtcactgtgctcggccatatatgtcagtttttaacacaagcatctctattttgattctaaccgctttcacatcagcttatgtaaagccatagaattaaattagcacatttttcttcactatcagttttacttgatttggatggggtaggaaaatatattatacaaacaggtagagataaagtagaatgtaataatttgaatgatttaggacaagcacaaaactaccaaaggaatttcaagctcatagtgctccctccccaaagccccccagctacctctgggttttgtattcactttctgatgtctacaggggtactttgttgttaatgtttgaggagcattaaattaggagatcataaaaattcaggagtgaagcaggtgagtacccagctaagaggttgactgaggccaggaaagtgagaaagggctgtgtaggaaggtgggtcctgaaacccaactgaatttgaagaaggcgagatacgaggaggattcattcattagtgaacttggtgttctttatgttgctcctttctgttttacctcagacctgagtttgggaggtgtccttttatttcctgttgatgataaagaatcaagaaacaaagggcaagatttggtaagtaaaacccatctcttctcagaactacaagtggactcacatcaacttctcttgaagtgtcccctgccccaattggcctctctgctagtgtattagtttgttagggctgccataacaaaaagacacagactaggtagcttaaacaacagaaatgtatttccttatagttctggaggccgaaagtccaagatcaaggtatcggcaggtttggtttctcccgaggattctctccttggcttgcagatggcggtcatcttgctgtgcatgcacaaccctggtgtctgtgtgtccagatttcctttcttataaggatagcactcagaatggatcaggccccaccctaaacccttgttttaacttcattgcccctttaaagactctgtctctaaatacagtaaacatgaggtacggggggttggggcttcaatatatgaatttggggggacacagttcagcctataacaagcagattgggccatagtctccactgtacttcccctgtccccaggcttccatccatctgtccccggagcaccgtccagatagcagatcccatcttaagtacgaggatttctatttgtctttttatcctcagtaccctacatagtactagctcataagaaatgctccataaacatttactgcatgagtaagaaggcatgactcagaactctgacggtttcatttcttactatgtgaaaatttctatgaaagattgtgttttctagtcagccataataaagcaggagagaggaactaacacatatgtcctctgcccacatcagaatccttttgcatcttaggcatcttgggatgcctgtagtgagtttgatttaccccacctacctggctttctccaaggcctgggttcatgttcagattttaagccagaattaagaaatttcaaaatcaggccaaaagagaggctcatccttttgaggttgctgtctatgtgactgtgttaggctgtttttgcactgtgataaaagaattccctgagactgggtaatttacaaagaaaagagatttatttgctcatgcttctgcatgctgtacaggaagcctgatactgacatctgctcctgctgggggcttcaggaagctcacagtcatggtggaaggcaaaggggaagctagtgtatcacacatggcaagagcaggaacaagagagagtgggggaaggtgccacactgctttaaataactagatgtcatgtgaactaccagagcaagaactcatcaccaagggtatggcattaagccatccatgagggatccaccccatgatccaatacctcccactaggccccacctccaacactggggattacatcctaacatgagatttggagggggacacacatccaaactacacagtgactaacagcaaagtggtttctgttgagtcattccttcagtaatttctaaaatgctaaaaaaggagaaaagtaaagtgtctgtgcatgagaaactcagaatccagtgattcaggaaaactgtttacagggagtagagcaccatgtctatgatatgactgtggtgatgtcatcccggaagctcccttgacactctccagctcgcccacttaggttaggatggttgagagatacttggcattttgtcctcatgggaattgttcgaacagagatggaatgactgcttgtcctgggggttgtggagctgactcaggcatcaaagggctgggatacaggagcctctaagatcttttccatgcctacaattcagaaaaattctctttttttttttaacccttgagagcttttggaaagtatatgttttggactcattctctggttttaaagtattttaaaaagaagaagaaaaccctgtataaagtgaccacaaagtaagaattatgacgggatatgaagtcatacatatagtaggacattgctgttcaggcatagcatccgaaagagacagagccaagcccaagtgacccatcaagggctgtgccgcctccatgggcggtcacttggttgagtgtggctgtttcatgttgggttggtcatctaatggtggttctttccagttggccttgattgtggctcagcatcgtgatcgttccaatgtcctgtctggcattaagatggcagccctagaagagggcctgaagaagatatttttagcagcaaaaaagaagaaaggtaagctcttccacctgtgctcaagagtagatgaatttgtttctaggcatgtgatacgacttttgaagggaggtaagaaatgtcaagatcccacttaatatgcacggtaaaggcaaaccacagaagtgatcaccccaccgtcttgtagtcatatagccccttgtcctttccaaaacacttttaataccggttatctctgtaggccgtctccatcccccgggtatttttatcgtgattttacagatgaggtggcagaggactagacatgaagcaacttggtcatatgtagttggtaaatgctgtttatttaatctcctcttggagagtcacagttcccaataacagacagttcttcgacaaaaattgagtttagttttgtttcgaaacctagtgtgtctcagagcttattgaattgattggcttgttagagaatctttgcttattttaattttgcctccaccaatcataatctatttccaattgtatgtatttccagaacttgtaggtccttgtgttcaacagaataatttaatttttcttactacaattcttcccccggaatatttttgacattataattatgggctttgagggagatagtcaataataattttctcccatgtgtattttatacccatcaatcaatttttgatgagtgaagacatgtgttcttctcttcataatagcaagtgttcatcttccacgtattggacatgccacgaaaggttttaactggtatggtactgagcgacttattcggaaacatctggctgcaagaggcatcccaacttacatgtatccttttgtgatcttcattgtgtgttctcccaacccaagagggaaaatgtgttcattttctggtgtcagttcttaatccaagaccaagtttcttcctgccacagtctttactttccccctcttcagtgagacaaagaaagaagcactttctaacttgtgtgtatcaaatatgtacacccaacaggatcaacacatccaagcatttctggatgccagcagataaattaaaagatacatgaaggggagaattaattgagcaattgttaatttggtaacatattgagtctgtcacatcacttctctagagatccttcaggtctgtggaacaaggcttaattctaagaacttcacactgttcattttaatgaacagttaagcaaacaaataagtgaactattttattcctgaacctttttgatgtattgttaaaaagcagtatgaaatttattttaaccatgaagtcatgatctactttagctagactagcgttttcttctaatgacctccttgctctataagttagcatattttgaactattatattgagtcccaaaattactagagaaagcagaattgaccccaagtgctataatcacacagaaactccatctttttacatatttgactgaaattcactcagtgatggtcttcaagatatttaaatcactgtaaaaacttagagaagccagcttttatgtgcttgcacaattcgagcagtatctaaagagttttagtactctgaaaacaacagcagcaataagtactaatattgaaagtgtttatgatatcgtgagagaattaaagcatactacttctagaacagttatttcaataattactagagaactagtcgttttggtaaagttggtttaaagtgatgacatgtatcttccttgaccatccttatcagatattattttcctagaagcaagtctgctgtccttcattcacagtcttcatcttcctcctcaagacagctggtgccttaagaattggcccagcctcagatcctgtctttagcaaccagctaatatttacccagaggtactgcaatagagtatttcaaaatggaatcaggatctggtgggcctcagaaattgtctcttttctgagtttcagtttggttctcctggatgttttgctctgttttggtacctgtaatatagggaaacacaactttttttgggaaagccctttgaccccagcttgctagttgcataataataaattttctgttcctaa